European Patent Application EP 4 643 637 A2, published November 5, 2025. Title: HIGH TEMPERATURE SEED GERMINATION. Applicant: Rijk Zwaan Zaadteelt en Zaadhandel B.V. Application EP EPPCT/EP2015/071082, filed September 15, 2015. The sequence listing filed with the application follows.

SEQUENCE LISTING (69 sequences)

SEQ ID NO: 1 - DNA, 3900 bp, Lactuca sativa
  misc_feature 1..3900: note = source = /organism="Lactuca sativa" /mol_type="unassigned DNA"
  source 1..3900: mol_type = genomic DNA
tcgattttgagactgattttcaatgtttaagaaagtcactatattaccataaaatttcgattttgacatgagtttttttttctcaattatatgattaaattttcaattctgttgccatgtcaaccaacagagcgattcaggagatgttattatggtttagaagctcgatttgtacaacaaataaataaaggtcaatataattgttcaaactcacttgtaagtcagtgaaaagggcatagtcaccattttaggagatgttattgcagtttagaagctcgttgtttacaacaaataaatgacaagacaatattgtgatgtggaagctatgcccgatcttatgtggtaggattgagtttcaaatatagggtttgcatcgaacccaatttcacatatctttttaggtcgacctagtgggtcaaactcacttaaagttcagcaaaaatggtgtaatcgcccatttaggtgacactttttattataatgtttaatgtttaattcttgtcagagtatttcttcacaaatgacgtctgaaggtcaatctagtggttcaaactaacttaaaagtcggtgaaaagggtgtactcaccctttcaggagatattattgtggtttagaagctcgatttgtacaacaagtaaattaagacccctacaaggtcgatcaagaagatgtttagtgagtttgaaccactaaatcgaccttgtaggattctttatttatttattgtacaaatcgagcttctaaaccataataacatcttttggaagggtgtctatgcattttttgctaacttgtaagtgagtttgaatcattggaccgacctttatttaattgttgtacaaatcgagcttctaaaccacaacatcttttgaattggtcaattggttgatattgcaaaaaaattgtaaatgtagtgatataattgaaaagaactcggtgtcaaaatcaaaattttgtggtaatataatgactttcttgcaatttgaaactcagtgtcaagatcaaaattttggtaaacttagtgactttattgcaattcgggaaaaatggttaccgggagaacatagagaagtggtcatttggttgatattgcaacaaaattataaatatattgacataattaaaaaaaaaaatttatgtcaaaatcaaaattttatggtaatatagtgagtacttgtcatttgtcctttatgaaatcaacccttgaggctttaaatgaggttaccatatgaaattgaggatgcaacaaaccttgaggactaaaatcgtaatttacaaaactaaatatcaggcttgaagtgaggttaccatatgaaattgaggatgcaacaaaccttgaggactaaaatcgtaatttacaaaactaagtacatgcgataacaaattttgtttggaaaatgacatggatatcggatagtgttggattgcacctttgaaatttgaatctttatgtttttaagtagttatatatttggtaacatatacaaatacacataacataataaaattaagatgtaattttgtttctcttttttaaaatattcatacacaaaatcaattctatatcctctcttcattaaaataaaaggaaaactaaattaaattgggtgagatgaatattcactcaacagacaaaacttttcatttcttttctgaaacgaaaggaaaacaagactacccatctcttttgtatctatgattgtactaccacttctaatttcttttttatataacgacaacttcatgaagaatcctaacccatttcatctctcaatctcacttactttcttacatctataatggctatctcttcttgcctttgtcaccatcaattagcactcaaggtattgttgctttcccattctactgtatctacgtgtatctgcatatgttcaaacgaattctccttcaacattcatggtttatttgccatttttgcgatctgggttcgagttatttcacgttcttggtgctgaatttggttggttttgccaatttgtgtatttgcaaatgttgtaatcacttcacctttgcatattcatgatttgttttccaatttaccaactgggtatgattcattttgctttcttcgtatcaatttagttatttgtgcccatttcactctgtttatattgtgtgtttgcagattgaatcatcactttgcatatatatgttatgatgttcatatacttatataacttgtttgtttgtacttttcccccaattgaattggtttactttcccgttttcatgtttgaactcgattggcaatttagggttcatagatgttatctctttgttgtagattaacctcttaacgactgcatccaaacactcgaaatccacattcgctattaaacccatcaacaccgaattttacggaatacatatcggaaacaagctaagaaatcaatggagttttatgagaggatcaggagctataatcataccaaacgaaagcttcaatctgcgtcaaaaaaactcaaaattgcaagcatcatgtaatcctttcgtaccctttgtttatcatgagataatttatcgattaaacatctaaaactttgttaatcttatcaatttatagttcgattggatctttgttcatgtaggttttgctagtatgcaattagcgagtgatgcttttacattaggaactgctgctgttcttccattctacactcttatgatcgcagctccaaaatccgaattggtaaattttacaatgttataaagcaaacaaaaaaaagaaaaaaaaaaaggtatcgaaataactatttaatgctttttctttttcttttgactttataaaaacaagaattaatcttataaactatatatagatatttctttttgacataatacataaagaactaaactttaaacttacactcatgggactctgtctagctgatgtgagacactgaattgttttaacttgcagactaaaaagtgtatgagaagtagcataccatacgtagtgcttggggttttatactcgtatcttctatatctttcgtggaccccggatacatttcggttaatgttcgcaagcaaatattggctgcccgaggtaagaatttctgcccgaatgatttgataaatgataatagcgtatttttaaactttaccatggtttattttcagcttccgggtgtagctaagatgttttctaatgagatgacattagcctcggcgtggatccatttgttagccgttgacctctacgcagcaaggtatgagggtatttacgtcttttgcacagacaagatatcagtagccaatcattgtcccacctttatgggtgggatgaaaatttgtaaattatgtaccattgtgtataagtctggtgcatgtcaaacacaatctgatgcataccaaacacagtacatgaaacgacagtcgtactgattgaagttaacttatggttttgattggtggtaacagacaggtgtatcaggatggattggagaatgagattgagacgcggcattcggtttctctttgtttgttgttttgtccaattgggatacttgttcatgctatcaccaaggctttaattagtacatttagagaatcaaaaagtgagattcattgatgtttttatttttcctatcaagtgatggagcatttatttgttcaagtcttttaatctaattggttatggttttggtgtaaatctttacaattttaatcatgaatatgttgtaggatttgtcttaggggtttatgatagcattgacataattaactcttcaacattacacggaatcaaataaatctctaattccataaaacaccttgtaatcctcccttatcccaacataatctacaattccacttgtgccaataaggaccttttagtcatttcactattataagctttttatccacgacaagatc

SEQ ID NO: 2 - protein, 236 aa, Lactuca sativa
MAISSCLCHHQLALKINLLTTASKHSKSTFAIKPINTEFYGIHIGNKLRNQWSFMRGSGAIIIPNESFNLRQKNSKLQASCFASMQLASDAFTLGTAAVLPFYTLMIAAPKSELTKKCMRSSIPYVVLGVLYSYLLYLSWTPDTFRLMFASKYWLPELPGVAKMFSNEMTLASAWIHLLAVDLYAARQVYQDGLENEIETRHSVSLCLLFCPIGILVHAITKALISTFRESKSEIH

SEQ ID NO: 3 - DNA, 2000 bp, Daucus carota
  misc_feature 1..2000: note = source = /organism="Daucus carota" /mol_type="unassigned DNA"
  source 1..2000: mol_type = genomic DNA
ttggaatgggtgcattagtttatcagttcgtattgtagatttatgtttttataagggtgaaattttctggaattcataattaacaggttgaaattctgccacctaaatgtgtgttggactgatcatttcaggaactgaaaatgtgattgttgaatccttcttattcttgatcgattttctttatagccatcacagttaagtttgcaaaataatgaacaagtttgttcttgagaatcaaaatgccctcctggtttcaatcctaaagttggggcagtacttgccgagttggacatgggaattattaaagtatctatctttatactgtctcccaaatgcttatgatgaaaatcttgaaactgaatgcttagtaaattttcgtattatatggtgctggtacttggttgcttctcattaactgttacttccattctcgccttgtagaccgaacattcaagcttgactaggaagggcttctataatatcagcaagattcagctaaacccagttgctattgaaggcacaaacagtgacctttatggccaacatgtggtgctttggacaaagatgagaaaagaatggagttttaagagaggatcaatatctattgctggtccgactatggaaagatttgtgcttcacagaaaaagctctggagtgcaggcttcatgtgagccccctttctttaaatctaccaaacatttttacttgtgtctaattttgtgtagttatcacaaattcttagaaatatgtatcagttactttacctttattgatgaaagcacctgtgattttgaacaaatgaaatgcaatgaaatcttgatggtcaatgatgcaaaactatgcaacaaaatataatcgtgtataataaaaccaaagctttgatctgatgtacttttggcataaggaatgatctagttgtttgataggggtaattaaattgattgacatatatgcatttttattctaagcaactggttgagggtggttgtctggaacccagcagaggctaattatgccatagttcttgcatatacctgaccttgatgtgtatgacttaatggcagtcttttcactgtggccttgcagggtttacaaattctcaaattgcaagtagtgtttttacgttggcaaccgccgctgttcttccattttacaccctcatggttctggctccaaaagctactctggtaataatttattgagacatggtgactgctttgactgattttatgttcacaacttcacatatgtaatcagacatgaaaataatagaaacttgagccatgtgactaattatttgttttatctaccaaattcagactaagaagtgtattcaaagtgcagttccatatgttggtcttggacttttatatgcatacctactctacctctcttggacacctgatacatttcggttgatgtttgcaagtcaatactggctgcctgaggtacgtctcagactagcacaaacaaaagcttaagctttttactcgttaaaattattaaacattttgggaaattttttttgaggtaaaagtgatgattttggtccatctttggctcaatatttttattgtgcagttatctggtatagctaagatgttttccagtgagttgacattagcttcggcatggattcatttgttggctgtggatctctttgcagcaaggttcgtaagtgtttgaatgtgcatatacgtcagggtgcctgcagtccattaaaattaaattctcacagttaaaccattttctaattatgcaggcaaatatttcaagatggactgcagaattctgttgaaacaaggcattctgtttccttctgtctactcttttgcccgataggaatcttatcgcatgaaattaccaaagctctaaccacaggtggaagaactgccaaacgcgagatccattaatgcaaaaatgatcagctgacagagtatccattttcctatgacaaagatagtagaggcttttcttgctattagtgatttgttttcgag

SEQ ID NO: 4 - DNA, 2163 bp, Daucus carota
  misc_feature 1..2163: note = source = /organism="Daucus carota" /mol_type="unassigned DNA"
  source 1..2163: mol_type = genomic DNA
atggcttccctgtcttgcctctgcagttctcctctgtttcttaaggtacgtgttctgtgtttgctgttcatatagtctcaattctaatcatgcttggaaactcgttatgtgtttgctgttcatatagtttctgtttgtattcgttagattgttagaagatataatataatcctgataagcactcctttcaacatctcgaggttttgggagaactgatcacttgacataagtgtttgcatgatttattcccagggagggcggcaaaaccctgatttaaagggaaaactaacccagcagtactacagatcatagttataaataggtatcattcagtagaagaaaattatgcaattcagttaagcaattggatcatgaataaaaaaggacggtgatgagttcacttttcattgtagtttaggttttggcctttatatatgttgttgtcatagttcttggtattgaactccaggtttcagaaaagaatttcaaattctataagaatcttaaactgaattagttgtacgagttatgtgagaagttcaagtttgaatccagtagaagttcaagtttgaatccagtagagtttattcgctttgttaattggacatgtttttactaaaggtagtcggccttttgatcaatgatctatctccgtttatagtagaaaatataacagacttgatgtgaaatttagctaatagtttaaccttgctgtgatttctataatagtgaatagtcttcactcttcagatatcttgttggtgataaccttgtttctgctttaacattgtagaacgacgaatcaagactggctaacaaatcgttattagcctataccagaaaggaccggataacaacttattgtcttaatagtgtcgaaactgacccttttagtcgacatccacatagcataaagacaaagagatggagtttcaaaggaggatcgagggtgatcactggacccaatattcaaagatttgcttgttacagaaaaagctgtggagtttatgctttatgtaaattcctttttcacaaataactttgattgagaattttaatttactatgcataccctaagctgttatccttggtatcttctatatcgagaattcttcttatcctttaataaaaaaaattgccatgcgctcaatattgaactgctttttgtgaccttgcagggttgacaaatcctcaaattgcaagtagtgctttcaccctgggaactgcagctgttctcccctactacacccttatggttgtagctccaaaatctgagctggtaagcctaatatggtgacagcttttactgaattgcaaatactacgatccattctgaatccaaaatgttttattttctaatagttgagctaaattactgatatgcctgatgtttacatgcttcgatattcagaccaaaaaatctattgaaagtggcataccatatgttgcgcttggtcttttgtatggttacctactctacctctcatggacacctgatacaatgaagatgatgtttgcaagtgaatattggctccccgaggtgtgtttgaactgtgggaagaacacgcggtttttctaattgcagaaatactttgtttaaaaaaaatttaattaacatatttacattctgacagttatctggcatagcaaagatgttctccagtgagatgacactagcttctgcatggattcatttgttagctgtagatctctttgctgcaaggtccgtttctctccctcatttcccgcgagccttaactcttataccatgttaagtgaccaattctcccaaaatttcaagatgttgggggaggggcttacgaggatcatattttattctaacagttctaacatttgacgtattgtgatcctattaatcaggcaggtttatcaagatggactggagaacaagatcgagactcggcattcaatttccctctgcttacttttctgtcctataggaattatatctcatgtagtcaccaaagcactaaccaaaagtacagagtaatccagtaagtagcaagattcacttgtgcctaaagcatgcttttcatttgactacagaagtacaatgtttgttactgcagattccctggttttgcatttcacaattttagtcggcttttccatgatatattgctcacaattgctaacttctga

SEQ ID NO: 5 - DNA, 2028 bp, Cichorium endivia
  misc_feature 1..2028: note = source = /organism="chicorium endivia" /mol_type="unassigned DNA"
  source 1..2028: mol_type = genomic DNA
atggctttctcttcttgtctttgccaccatcaattggcactcaaggtattggttaatttccccttttactctctctatgtgtgtttgcatatgctcaaacgacttcactttcacgaattcatggtttatttggcatttttcgatttgggtacgagtcatttcgcgttattggtactaaatctggttgattttgccgatttaactaccggtgtcatccaatttgtgcattttcacatgtttttagctacctcacttttacatattcctgtttgtttgcgaatttactatctgggtgtgattcagtttgctgtgttcgtgttaatttggttgttttggctcatttgattctgtttattacatccatttctgtattgtgtgactgcagattgaatcattcactttagatatacatattatgctgtctgtaaatctattcgtttgtatcttctccccaattgaattggttcactcttccgattttgagttcggttagcagtttagggttcatagatgtttatgttcaaattagaaccatcaaaaggcttacatgagtgagaaatcttgaagatgttatatctttgttgcagatcaacctcttaacgagtccatcgaaacccacattcgttcttaaagccatgaacaccgaattttacggaatacatatcggaagcaagatagaaaatcaatggagttttatgaaaggatcacgagccataatcagaccgaaccctggaagcttcaatctgcatcaaaaaagctcaaaattgcaagcatcatgtaatcctttcgtatccttcgtttatcatgagataatttagcgattaaacatccaaaactttgttaatcttatcgtgttttagttcgattggatcttttttcatgtagggtttgcgagtatgcatttagcgagcgatgcttttacattaggaaccgctgctgttcttccattctacacccttatggtcgctgctccaaaatccgaattggtaaggtttacaatgttgtcataaagcaaagaaaattaaaaaaaaaaaaaaaaaatcattcaaatacctatctatatatcaatataattggaatttaagtgatgtttcttttttactcatttaaagtgttgaatggataaattggttttttttttcttttttgggtaaagtgtcgaatggtctaatattaattgtttaatattaattgtttaatatattaagtccattaagtgaaaaagaaaacagacgctaagtgtttacaaatttggtcgacattaatgcagacgaaaaagtgtatgagaagtagcataccgtatgtggtactcggggttttatactcgtatcttctttacctctcgtggacgcccgacacaatccgattaatgtttgcaagcaaatactggctgcccgaagtatgattttacacccctatagtttgctagatagccaacttttaaccctagtgatggttttatttgcagcttcccggtgttgctaagatgttttctaatgagatgacattagcctccgcttggatccatttgttagcggtcgacctctatgctgcaaggtaggaggacatttacgtcttttgcacaaacaacaaatcggaagctagtccatgtcccaccttcttcggtgggatgaaaaattgcaatttttctcccattgacttctgtgtacctgtacctgtacctgtacctgatgaattgtggttttgattggtggaaacagacaggtgtatcatgatggattggagaaggagatcgagacacggcattcggtttctctttgtttgttgttttgtccgattgggatacttgttcatgctatcaccaaggctttgataagtacatatagagaatcaaaaacagagattcattgatgggtttttttgtgccattaagtcttaaagcatttatgttatcttttaatctaatcgattatggttttggcagaaatgtttacaagggttggttatgtagacgctgtcatagggttttattatagcattggcataattaatgttatgcgactataa

SEQ ID NO: 6 - DNA, 1507 bp, Solanum melongena
  misc_feature 1..1507: note = source = /organism="Solanum melongena" /mol_type="unassigned DNA"
  source 1..1507: mol_type = genomic DNA
gatgaactgctgggcaccagcctcggtgtcattgagtacccgcagaaaccacactgcctttcttgctcttagagaaattataagtcaacgtattggtggatttggaaccaagcttagcagtggagggagttctctgggaggatcaagagtcattattcaactaaatcttcaaagaactctttcgcaaagaaaaagctctagggtgcatgcttgctgtaattactttcttacaaactccattctttgtgataaaatatctctggttttgaatgtttatgacaaagtaatcttaaatgtgtgcttaattaagttctcgctgtacttaagatttatcgtctcatccattcccccttttttttggttgttgttgtttatttggagagaaattgtttaaaaagctactactattttgcctttagttttaatgaattataaattactcaagtctaaatggtgctttgtgcatagttaagagtaaaacttgctataggtgctttaagagtaatcttcttcatgcagctgttaatgttccttgacccttctgtacagtttagcctctggttttggcagacttttatgccaacgactaacactggttcagtttttagctaagtttctatattcttttgcagggttgccaagttcagaaattgcatctactgctttcacagtgggaacagcagcagttcttccgttttataccgtcatggttgtggctcctaaagctgaactggtaagatttctatagtactttcagtctgaactccttaagcgattccttttctagtgtactagagatcaaacttggcactcaaattatgaattcaaaagaccttaaacacttatcagcttcagacaaagtagaacagttgggcacaacttcagtccttttatgtatatggaagtcactgctttatttaaaagagaaattgtaattgaacataatttcgaatgcagaccagaaaagcaatgaaaagcagcataccctacattgtgcttggacttctatatgcatatctattatacctctcctggacaccagatacaattcggctgatgtttgctagcaaatattggcttcctgaggtctgtgctcgactacataataatttgtacaaattgcatggtcgggatcttaacacttcctttcattcagctgtctggtatagctaagatgttttccaacgaggtgacgttagcttctgcatggattcatctgttagccatagatctttttgctgcaaggtcaatctttaggcgtctttatctttgttgggctatgcccctttgctttctttttgggacaacatgaggaggatgccactgttagacatctaactagagtatctcacttgaaacaggcaggtttatcatgacggattgcagaatgatattgaaacccgccactctgtgactctgtgtttgctgttttgccctgttggaattcttactcactgcatcaccaaagctctaactagcagcccagaaaagaaacagcataggactc

SEQ ID NO: 7 - DNA, 2919 bp, Solanum melongena
  misc_feature 1..2919: note = source = /organism="Solanum melongena" /mol_type="unassigned DNA"
  source 1..2919: mol_type = genomic DNA
tctacttgcttttgtcactctcaattctcactcaaggtgtgccttttctgcttctcctctattcatagcttgtaatatatgttcttcttcatttgtctaggtaattaaattggtgtttattgttctcaatttttttaattgaatacccatacctggtctgtatgttcaactgacacacaactgtttgtttagatctgaagttgctccattgctatatgataatgaaaaattcaatttgagagcacctaaaatgctagtgaaggcttcaggtagatactgcaatagtggagctagcattttcaccaagggtgttcatacttttagaacatatgggtgggtgggtgatttttgtatcaaggtatatatataaaaatatttatattttgaaaaagttttccaacgaaagatggttcacccttgggtgaatgtagttcgccccctggtagatagtgagcaacatctatgatttaaagatgtttttggcaatagagggtggggatggtggttttagtgaattgaatgtcaatctggcaccattgaattatcacttgttcgttgaattatgctatgagaaataaggcttagtgaatggcatttcatgctcaacacatattcgataaaattaatttatacttggtagttgaaacaaaaaagaaagaaagaaatgaggtttttctacgcactaaaaatgaccaagtttgaaaatacaatgaaatgtcattcctgctgaacgactatgctacttaccttagatggaaagctggacacctgctctgtcatcaaatatccgatgttatatcaggaggaaccagtttccatcctccatgcttaaaacaataaattctgacctttcaagtcaacaagttcaggaacgaggaaccaagcatagcaatgggtccagtttcctcggaggatcaagagtaatgcgtcagcctaacctccaaaatcttccacaaagaagaagctgcagggtgtctgctatgtgtaatcttttcttcgctgcttccttagtctttatcatttatttttagctctcattctgtgtcttgctactttctttttggataattcttgggaatcagctatacacagtcaggaatctggttatccatcttaatttacagtcatcacataatgttgcgaattaggttattatgacacctccctgccaactgctaacacatctgttagtttaccacacttgataaaaaaaatttattacaatgcttgttaactttgtacaaatactctatatggccttttcttaacacgtttggcttaatatccacacctactttcctccttttagatgaaccagggaaaacaaattcgaaaaagaaaagaagttgtagaagtacaacaatttgctgtcttccttcatctggttgaaactttgatatctcccaccctgagtcacatgttccattggaatcttgtttccctcattacgttgctggattttccatctcatgtcaataaagactatgcttacttgctcatgtagatgtgtaaattgctagtctcccagatcttatcaagtgacagttttgatgtattgtatatggaatatcaaactaaatatcaaattgatctactccatttgattataaatccatacgtatatgtataaatacttatttatgaagcttcttattgtttactctctttgcaaatgttgcaagtatcacctatttgaacttttgggacaactgatgtcttatttttacagggttgcctagttctcaagtagctagtagtgtctttactctaggaacagcagccgttcttccgttttacaccctcatggttgcagcacctaaagctgaacttgtaagttatctcagttctgtaaagctacattctatttttgaaaattttctagagtaaaccctctgggtgtattttcaacttaagaagctcttgtttatttttttaaaattggaagacataaaaagtgttacttgcaaagttctctctccccgtgtcatgcacaaaagtagaactcggggcatgatttcagttgtattgatttgttatctaattgcaagatacttaatttcgtgcctttccgagatatactgtaatagggcataattaaatacttaatgcagaccagaaaattgatgggaagtgccataccatatgttgcgctcggacttctgtacacatatctgttgtacctgtcttggacaccagatacaatccggctaatgtttgctagtaaatactggcttccagaggtttgttcttgtgcttagcaaatgatggttgtcatcttgtgctgattctataattagggttgttgacgtttcattctgttcagctctccagtatagcgaagatgttctccagtgagatgacactagcatcagcttggattcacctattggctgtagatctttttgctgcaaggtctctctttctctcgcacacacactttattgtatgtgttagattgttccatgctagttgaggaaatgggtagttgtctccttgttaggtgttgccatgttggacaatccgcattttatgagctagtgtttcgggtggtatcagactcatcacactcttggtttactcaatgtttccacgcgccagatgtccggtcaagggcatacagggagggtggaggaaggatgtttggttgtccgactgttctcgcatgtttgtgtagccagttgtttgcttgctaatcctattgggttgaggaaaatggaggaaggtgctttgttaaactattctaatgctgttttttatttgaaacaggcaggtttatcatgatggtttgcaaaatggtattgaaacgcgccattctgtgtctctctgcttgcttttttgccccattggaattgttattcatctcctcaccaaagctgtactaagtaatgcggaaaacatagtgcctagaactcactgaca

SEQ ID NO: 8 - DNA, 3000 bp, Solanum lycopersicum
  misc_feature 1..3000: note = source = /organism="Solanum lycopersicum" /mol_type="unassigned DNA"
  source 1..3000: mol_type = genomic DNA
caaaaaggtgtaaagtagcaccaaggagtaagtgcttaaacaactttccgtccaaatagaggtgtgtggtcggatttggcaaattctcaactaacatcacaaaatgcaatatattattaacattattagtcacttcatgatttctttatttgcaccaaactttgagttgcttctaaagctaaaaataaattatactttttgttgcttctgtttttctcattattgttgcaacttcaacaacaataaagcatgtacttctcttcttcttcccatgtttcactcaaggtatgctctttctttctttctgcttctatgtcttgctctctgtttctgttttagctctgatatgttttttgcctctcaaaagggcctccacagtcatccactgtttcttgctgggtattgatatttagttgagttgtttgatcagtttataagcttgatatttagttgagttgtttgatcagtttataagcttgaacgaacgccctcgtgatgctttaggaagatattgttagcccacaagttagggcttattcccactgaaaaatagtcggtacatattttgattgaatcgatgagaaaaagaaaaaagtaataatcttttagtatagaaaaattaggaagtttcccactattatgattcgtagtgggaaacgcttgtgtttctagtaatgacgtgggaatagcctcttttcgaaatacaagaagtgtgtacagtgtatatatgcccactctttccctctgctggcactagcagaagtcctttttgcacagggtaagctcttaggttcacattattgagttacaggcaaccagaaatggaaatttacgctaacttcttcgttggaagagatgttggcgaaggccacaaagctagaagggcattttgtcatcttaaccaacgtgcacgtgcaatgatgtgaaatccaatatcttcgtctacaattacttgtcgtaacacgtttctgctctaagactttctctcaacatatctgtaagcagggagtccgcattcactattaagcctacatagatgtggagattattgaagattgaggcactagctaaatgaaggtgttttagatcaatgtgaggtctagcacacctttcggaataggactacaaataaataaggttttgcaatgcattgaacctgaacaagttggaggctacaacgaaatttaactgcttttcacgcagtcatttttgtttatcagtctataatttcatttcctgaaacgaaccattacttgttgcagatgaactgctgggcaccggccttggcgtcaaaagtccctctgaataccaggagaaaccagactgcctctcctgctcttagacaaatgaagtctgaccttttaagtcaacgtattggtggatttggaaccaatcttagcagtggagggagttctctgggaggatcaagaatcattactcaactaaatcttcaaagaactctttcgcgaagaaaaagtcctatggtgtctgcttgctgtaaattactttcttacaaaccccattctttgtaataaattatctattgttttaaatgttcatgagaaagtagttttagatgtgtgtttgattgagttattgctgcagttgggaagtattgtctcattcattgccctttttttgtttatctggagaataagattgtttttaaagctaatcttctgtacagtttagcttctggttttggcagacttttatgccaactactgacattggtcaagcttttagttgagtttctatgttcttttgtaggggtgccaagttcagaagttgcatctactgctttcacagtgggaacagcagcagttcttccgttttataccgtcatggttgtggctcctaaagctgaacttgtaaggttttttaagtactgtcaatctgaacttcttaaggatttcttttccagtgtactgaagattaaacttccactcatattatgaattcaaaagatttttctaaattaaacacttaccagcttcagacaaagtagaacggttagggcacaacttcagtccttgtcttgtgtatatgaaagtcattgttttatttcaatgagaagttgtaactgaacataatttcaaatgcagaccagaaaagcgatgaaaagcagcataccctacattgtgcttggacttctgtacgcatatctattatacctctcctggacaccagatacaattcggctgatgtttgctagtaaatactggctcccggaggtctgtgctcaaccacataataatttgtcaaaactgcattatcgggatcttaacacttcctttcattcagctgtctggtatagcgaagatgttctccaatgaagtgacgttagcttctgcatggattcatctgttggccattgatctttttgctgcaaggtcaatctctaggcatcttatctttgttggcctatgccccttcgtttttttcttttgtataacatgaggaggatgccatagttagacatctcacttggagtatttcacttgaaacaggcaggtttatcatgatggattgcagaatgatatcgaaacccgccattctgtgtctctgtgcttgctgttttgccctgttggaattcttactcactgcatcaccaaagctctaactagtagcccagaaaagaaacagcataggactcattaaccaatgttttaggccttcttatgttatccgtaaatgatcagccagcgcgtgaacttatgagcaaagtgtaaaggttttaagtcaatgaatacataagctatttcaataacttgtttctaagatggatgaatgtacaagatttcttcctttagttccactccaaacttctgatttactgcatccttaactaagcgtatgagctcaagcatgtcttgagaagttgcagaaccacaatttatgaaaaagttggcatgcttgtttgagaccatggctccaccaactctcaaccctttcaacccacttttctctatcaattctgcagcagaaacacccatagaa

SEQ ID NO: 9 - DNA, 3400 bp, Solanum lycopersicum
  misc_feature 1..3400: note = source = /organism="Solanum lycopersicum" /mol_type="unassigned DNA"
  source 1..3400: mol_type = genomic DNA
taaacgtgagggaccatttttgtcatttaatttggtaaaattttagttgtatttgaagtcggtctgtttcactcttatatgagaagagaattcatcaagagggccagggctcatgatttatcattctgttggtgaaacctctcattactgtacttgcaatgtttaattttattttccagatgccatttttgctataattcttattgttgttgctcgcaattctcacacccatcaaccatggccttatcttctacttgcttttctcactctcaattctcactcaaggtatgccctttctctgctactctctattcatagcttgtaatataagtttttcttcattaaattgctgtttattgtttgttctcagtttttttaattcataccccgtatgtatgttaaactgatacacacattatttgctacttgtactgtgtggttagatctgaagtttctccgttgctatatgaatacattgaaattgaaaatgaaaatttgagagcaattaagatgctagtaaagtcttcatgtagatagtgctgagcaactatctatcatttgaagatattttggcaatagggagtgtttggaagaaaaaactttgaagaatgaggtgctagtgtttggaggtttagtgaattgaatgtcaatcaggtaccgttgaagtctcaatgtcatttgaattatgctattagaaattaggcttggtatattgcatgccaagcaaatcttcaataaaatttatctatacttggtaacggaaaaaagaaaatgaggttttccaactcactaagcactaacgagtttgaagctacaatgaaattccaaacctgctaaactattgttttattagaagtaatcaatctctactacttactgtagatggactgctggacgcctgctctgtcatcaaatatcctatgttatatcaggaggaagcagcctccatcctccacacttaaaacaataaactcaaaccttttaagtcaacaagttcataaacgaagaaccaagcatggcaatggatggagtttcctcggaggatcaagagtaaagtgtcagcctaacctccaaaatcttccacaaagaagaagctacagggtgtctgctatgtgtaatcttttcttccactgcttatctttatttctcaactcgtgtcatgctacttcctttttggttcttttggataattcttgggaatcagctatgttcggtcaggaatgtggttatttacagtcatctcataatgattcgctttaggttattatgacacctacctgccaaaacatatgttaatcaacaaactgaattcaaaaaatctgttacaatgcatattaactttgtacaaatacttttatgtgcccacttggcttaatgtccaaacctgttatcctcctattagatgaaccaggaaaaacaaattcaaaaagaaaagtacttttagaagtataacaatttgctgtcttctttcaatctggttgataatagaaatatctcccaccttgtccaatgttccgttgaaatctcgtttctctcatttcgttgctggattttctatctcatgtcaatgaaagaatattcttacttgctaatgtacatgtgtaaactgctagtgtcttacattataccgaaagacagttttgatgtattgtatatggaatatcaaactgaatatcgaattgatctatttgattataaatatatatgtatataaatatttatacatgttttttaagcttcttattgtgtactctctttgcaaatgttttagtgtcatctatttgaacttttgggacaactgatgtcttatttttacagggttgcctagttctcaagtagctagtagtgtctttacgctaggaacagcaggcgttcttccattttacaccgtcatgattgcagcacctaaagcagaacttgtaagtaatctcagttctgtaaagcaacactgttttttttattttctagagagtatgccctatggatatattatcaacttaggaagctcttgtttatttcttttcttggaagacataaagaaaagttacacatgccaagttctctctccttatgtcatccacaaaagtagaagtcatggggcataatttcagttgcattgatttgtgatctaattgcaagatactgattttgtgcctttccaagatatattgtaatatagggcataattaaatacttaatgcagaccagaaaattgatggatagtgcaataccatatattgtgctcggacttctgtacgcatatctgttgtacttgtcttggacaccagatacaattcggctgatgtttgctagtaaatactggcttccagaggtttgttcttgtacttaacaaatgatagttgtcatcttgtgctgataccgtgatttaggctgttgacatttcattctgttcagctgtctggtatagcaaagatgttctccagtgagatgacattagcatctgcttggattcacctattggctgtagatctttttgctgcaaggtctctctctttctatctcaaaaccacacttcattattgtaaatgtgttggattgtccgtgttagttgaggaaatggccatttgtctctttataaggtgttgacatgttgcacaatcctcatcttatgagctagtgtttggagttgtgttggagccaggcggtaatatttggttgtcctacactagttgaggaatggactgttcttgcctcatataatcttggccatttctcaatttatgagctagcttttaagattgtttcagattcaaggccatttcgttaacagtatgtttgtgcagccagttgttcttttctgatcctattgggtcgaggaaaaaggaggaaggtgccttgttaaactattctaatgctgttttttatttgaaacaggcaagtttatcatgatggcttgcaaaatggtatagaaacgcgccattcagtgtctctctgcttgctattttgccccattgggattgttattcatctcctcaccaaagctgtactactaagtagtgcagaaaaaacagtgtttagaactaactgacagagattcaacaattgtttcctgttaacgactaatgtaattgtgaacaaaagggtaatcttcattcaactacgtaaagtgtgcaaatttgtatatcattgatccaacactgcttgaagcattcgaattgatgagctctccttatatttttcagtaaatctaaattctttttagatggccgaatgtcagttttctttcttggatcgttactcctgccaaataaagaaaacgtttcttcttctccaatccaattactgataggatgcaaataagaatttctcctctcatatttgccataaacattgcctataattgacttctaagtgacataaagttgaaatttgttctaat

SEQ ID NO: 10 - DNA, 2375 bp, Capsicum annuum
  misc_feature 1..2375: note = source = /organism="Capsicum annuum" /mol_type="unassigned DNA"
  source 1..2375: mol_type = genomic DNA
gataccctcttgatagtttaggttgatattgttaacccataggttaagggtacggacgtgtaaataacctctttgcaaaatacaggggggagtggggcatatattgccccctcttccttctgccggcacaagaagagatagtttgtgcacagggtaagttcttagaggttgatcttattgagcaacagacaaccagaaactggagcttacgtgaacttcttcaaggaagagatgttgcagacaaagggcacaaagcgaggtatctattccttgaggaagaagggcattttatcatctagacagacgtgacacgcataatggtgtgaaatctaacaccttcatcttcgatctctcgtagcaacacattttcagagctaagaatttctctcgacatcattctttttatttaagtcattaatattacaatctggaagcagggagtccgcattgactattaggcctacatagatgtaaagatatttgaagattgaggcatgctagtgtctgaaggcctagcaaattgaaggtccattagatcaatgtgaggtctagcacaccttccggaataggactataaagaaataaggttttgcaacacattgaaccctaaacttggagggtacactgaaattcaactgcttttctggcggtcatatttgttttacccatctagaatttcatcatctgaaattaaccattacttattgcagatgaactgctggacaccagctttcgtgtcaaaagtcccgctgaatacctggagaaaccagactgcctcccttgctcttagagaaatgaagtctgaccttttaagtcaacatattggtggatttgaaaccaagcatagcagtggagggagttcactggcaggatccagagtcactattcaactaaatcaccaaagaactctttctcaacgaaaaagctttagggcgtctgcttgctgtaattactttcttacaatctccatttctttgtcataatttatctctggatttgaatgttcacgataaagtagttttaagtatgtgctttaagttattgctgcagttgggtttagtagtctcatcaatcgtcttcttttttttatttggagaataaaattgcttaaaaagcgcatattttgtcattagttttaatgaattataaagcactgaagttccaatgatactgagtgtaaaataaattagagttttaacagtaatctcccttcatgcagctattaatcttccttgatccttttgtacagtttttcttattttggcagacttttatgccaactactaacattagctaagtgtatcactggcaagctcttagttaagtttcttattcatttgcagggttgccaagttcagaagttgcatctactgctttcacagtgggaacagcagtagttcttccattttataccatcatggttgtggctcctaaagctaaacttgtaagatttctaaagtgcttttactctgaactccttaagcgatttcatttccagtgtactggagatcaaacttggcagtgaatttattaattcagaaggcgttcttaaattaaacactaaccagcttcaaacaaagtagaacagttggtacacaatctcagtccttatgtatatgttttccattcagtgctttagtttgatagtattgaattataacatgctgattttggcaaaagatgtaagtcattgctttatttcaaagagcaagttgtaactgaaaaaatttcaaatgcagaccaaaaaagcgatgaaaagtagcataccctacattgtgcttggacttttgtacgcatatctattatacctctcttggacaccagatacgatccggttgatgtttgcaagtcaatactggcttccagaggtctgtgctcaactacataataatttgtacaagttgtatggtcgggatcttaacacttgcttccattcagctgcctggtatagctaagatgttctccaacgaggtgacgttagcttctgcatggattcatctgttggctatcgatctttttgctgcaaggtcaatctctaggcatctatctttgttgggctatggccctttgatttctttttgggacatcatgtggagggtttcacttttagacatctaactagagtatttcacttgaaacaggcaggtttatcacgacggattgcagaatgatattgaaacacgccattctgtgtcgctgtgcttgctgttttgccctgttgggattcttactcacttcatcaccaaagctctaactagtagcccagaaaagagacagcgtaggattcattaaccaatgttttaggccttcttatgttatctgtaaatggtcagccagcatgtgactatcagcaaagtgtaaagattttcagtcaa

SEQ ID NO: 11 - DNA, 1510 bp, Brassica oleracea
  misc_feature 1..1510: note = source = /organism="Brassica oleracea" /mol_type="unassigned DNA"
  source 1..1510: mol_type = genomic DNA
agtttctgtcaaagagttcgtgaatcgaatcggagatggctttttctcagcctttgtcttcttcgtctctctcggtatttcgctttttttttagtttactccaaaatatatacatctgtaattattgtatatgttcatgtacacttgtttgatattgtccgattagtttctgtgtcgagctttacttactagtactcatatagcttagattccttatccttaagaatcaaatcagccaatcgatgggttcgcttgagttcacttgccctgtctctgtctgaaaatttcagattctgtgagttaaagtcgttatcaagtttttgttttttgttttttaatcagattagattcatttttttggtggtacagatgacgaatcggagctttgtagctaagagctcggtgacagcaagtctttctcttaacaagtctttaaagattcgattccataatcgttggagcttcgacggaggatcaagaatcgttctgttccccagtgtatcatccgattcgtcctcccttgttcacaagaaacgctcctgcgtacgagcttcatgtaatgtctctttttaactgaaaacattgaagcctcaaactttgtcgagagattctagttagctcttgtgatttcagactaaaaacatgttgatgttcagggatggctacgtctcaaatcgcaagcagtgtatttgctgtcggaacaaccgcggttcttcctttttacactctgatggttgtagctcctaaagctgaaattgtgagtccttttctttgttgcagtcttacaacttcttttgcagaactaaagaggttcatctgaaattgactttttttttcaagaaagaaattgaatatatgtgtttctttcagatttacaaaaaaaagtgtctctcttttgtgcagaccaagaagtgtatggagagtagcataccgtatgtcgtcttaggcgtattatacgcgtatttgttgtacctttcttggacacctgaaacgctcaaatacatgttttccagtaaatacttgttgccagaggtttgttttcaatacatactgtataacaatgtttcatagtagctactaaatgttttcctctctctcttttctttggtcatttgcagttgtccggaatagcgaaaatgttctcaagtgaaatgactcttgcttctgcttggattcatcttcttgttattgatctttttgctgccaggtatgttacaattttcaggttttggtttcaatcaaaagtctaaaacatgtttcttataacacatgttttgtttgtttctatgcagacaagtttttaatgatggcttggagaataagatcgagacgaggcactcggtttcactttgccttctcttctgtccggttggaatcgtttctcatgtggtaaccaaagctttaaccaacagttctacatccaacaccaacaaccagtgcaagtaaactgatcattgtggctggtctctcatcactgtctttcttaactgcttataaagatttttgattg

SEQ ID NO: 12 - DNA, 2169 bp, Apium graveolens
  misc_feature 1..2169: note = source = /organism="Apium graveolens" /mol_type="unassigned DNA"
  source 1..2169: mol_type = genomic DNA
aactcatatctttgtccctgtctacatacatatgatatatagatatgtttatgaccaagttgtctttatgacttttttgcaatgacctcaggatttctttaattatgtctactaccagacatatatgcatatgaatgtcaagagtgaattgaagaattgttggtggatttgggtatttgttatgatatgtctcttttgtttttgactgatctgcggtgattctgcaattcttcttctcagtttgtattgtcaattggtgttctttttaaggtggaatttgaataaccagtaggttgaaaattctaccaatacattatgtgctggactgatcatttcattcaggacttgcggatgcaattgttgaatccttgttatttctaatcaatttttctccatagccctcatgcctaagtgaaaaaaaaaactcaatttgttatgtgaaattcaaaatgtcccttttgtttcaatcctgaagtgggaatgcagttgccaagctgcgcatgattgaatctttttagaatccccatatgctgatatagaaactgaatgattagttgattaataatattttcttattatttggtattgtgatcgttcgttggttctttatttataacttgaacttgaacatgaactattacttaacttcatttctttccttgtagaccgaacattcaacattgagtacgaagcccttatgtaacatcggccagagtcggctgaacactgttgctattgaaggtataaacagcgacctttatggacaacatctggttctttggacaaagatgagaaaagaatggagtttcaagggaggatcaacatctattgctgttcctactattcaaagatctgttctttacagaaaaagccttgaagtgcaggcttcatgtaagccccctatatttgattcctctaagcacctcaatttgtttctaaagctgagtagttaccgcaagttcttagagttaatatcattaattttgttctatgcgacaattagtcgtcagcatctatgatcccttacaaataaatttatctagatggccaatgatataaatctatgtaacagtgtgaaatgatgaactggaaacaaagctttgatctgatgtaattttggcgcaaggaatgatcttagttgtttgataaaggcagttaatgtgaccgacatgtagatatttttattctaagcaactggtggaagttagttaggaacctagtaagggctaattgtgctaaattacttgctgttgcttaacttgatgtgtacaaattgttgctaaaattgaaatttgcaagtctgtagcattttgactggctgtcttctcactgtgaccttgcagggtttacgaattctcatattgcaagtagtgtttttacattggcaactgcagctgttcttccattttacaccctcatggttctggctccaaaagctaacctggtaaaaatatttgttggaacatggtgactgctttgactggatctaatgttctacttcatatacataaccagatttcaacctcttaaataattacgccgagtgactaatagttttctttttatactaaatttagactaaaaagtgtattcaaagtacacttccatatgttgttcttggaattctgtatgcatatctactctacctctcttggacacctgatacatttcggttgatgtttgcaagtcaatattggttgcctgaggtgcgtttcacacaatcaaaaaacaaaagcttaggctttcaacacctagtttttattctgaaacaatttggaagttgtttttgagatgaaacttatgattgtggtccatcttttgctcaacctttaaactgtgcagttatcgggtatagctaagatgttctccagtgagctgacattagcttcggcgtggatccatttgttggctgttgatctctttgcagcaaggtctgtaagtgtgtgcatatgtgtgattctttttgcagtgtattaatataaatttctcacagtagccgttctgttctgcaggcaaatatttatagacggactgcagaactacgttgaaacaaggcattccgtttccttctgtctactgttttgtcctataggaattttatctcatgaaattaccaaagctctaaccacaggtggaagaaatactaaacgccagattcgttgatgcaaa

SEQ ID NO: 13 - DNA, 2025 bp, Apium graveolens
  misc_feature 1..2025: note = source = /organism="Apium graveolens" /mol_type="unassigned DNA"
  source 1..2025: mol_type = genomic DNA
ggtaagtgtcctgtgktcatatagtttctattctaattgcgttttagtttgtagctatttttctttcttcgtttgtctacttgattaaatcttgtgaaggtgaattcaagtcatatttaaaaaaattgaatactaagtagaattattaagtactttagtatttacctttctatctatgttcatattgctctcttggatcctagttggatattatgtttctatttgtgttcatcaagaaagtgtttgcatgatatatatttttgtacagggtggcaaaaacccaaacttttatgcgaaaatttcgaaaaactgtatacagatcatcacagtcagcagtactacaaatcagtagtttcaaagttacaaattaactggaggaataatacaagtcatttaaacagttggatcatcaataatagtggagtgtgatgattttaatctttttattacagttctggttttagcctattgatgatatgttggtgtcagtttgtcgattgaagttttaagggtcaagtctactggaatttgtatgatatcgactactttgtaaattgaaactctggggttcaaaaaagaattttgaaatttgaactctaaaatgattttaatctgaatcagtttaccccagttgatttgctttattggacatatatatttactcaaggtgtttggactttgatctatccaatcctatatagtacaaaaatatgctgaattttacctttaaagcgattgcttaaatagcgatccttatgtatccctcagatttttttgtctatagttaagttcttgtttcacaggtgaccctggaataaggatgctaataaccttcatgtttctgctttaaaactgtagaatgacgacctaagactgactaacagattattagaagcctgttttagaaaggaccagttaacaacatgtgctcttaaaagtttcaaaactgacccttttagtcgacatccaccaagcataaagacgaagagtagaactgaatggagtttcaaaggcggatcaagggcaatccccggaccaaccattcacaaatttgctcgtaatagaaaaagctgtggagtgtatgcttcatgtaagttcattttccagaaataatttgatagtaaattttaatttgctatgcatatcctaagttgttatacttggtatcttttctctttgaatttgttcttatcctttcatatacaattgtcaagtgttcatgatctaactgctcttttatgttgcttgcagggttcacgaatcctcaaattgcaagtggtgctttcaccctgggaactgcagctgttcttccatactacactcttatggttgtagcgccaaaatctgagctggtatgcttctatcaccaaatgcggtgacagcttttattgacatgcaaatagtaattaggcccaatctgaaactaaagttttttattttctgaaaattgagaaaaacgactgatatgcatgtttacttgctccaacaatcagaccaagaagtctatcgaaagtggcataccgtatgttacgcttggtcttttgtatggttacctactttacctctcatggacccctgatacaatgaggctgatgtttgcgagccaatactggcttcctgaggtatgtttgagtagcttgtgggaaaaaaatgtggtttttccatttgtagaaacgctttgttgttaaatgaatttaatgaaccaaattatgttgttacagttatctggaatagctaagatgttctcgagtgagatgacactagcttctgcatggattcatctgttagctgtagatctgtttgctgcaaggtttgtttctctccctcatccatgtgtagctttgtggtgggagacttgccaagttctaacgtttgacattttctcatcctatcaggcaggtttatcatgatggactggagaacaaggtcgagacacggcattcaatttccctttgcttactcttttgtcctataggaattatatctcatgtagtcaccaaagcactaaccaaaagttcaaagtaa

SEQ ID NO: 14 - DNA, 2000 bp, Spinacia oleracea
  misc_feature 1..2000: note = source = /organism="Spinacia oleracea" /mol_type="unassigned DNA"
  source 1..2000: mol_type = genomic DNA
gaatggggcatgaaaacgaagtgatgacaaaaagagacagtggcgcactgtcatccctcccatcttttcttccttcaatggggaacaaagttatcttccttctttagtagtgatgatgatgtcaaatcaatttacatctaaacctaatcatcaacataaattcagtaattaagcattgttcattcattatactttctgggtcttttggaatttctgggtgttttttgagctcttctggtatggctttatcttcatgctttgcctatcatccccagatctcttccaaggtacccactctttttttctcttcaattcttttttccaataacaatttgtccaaattttgtgagtatcaaattgtttctggtttatattgagctcaaaattttgatttgattgcctttatattataaacgtgtgcatagttctgctggatttcatctgggtattgttcaaattaattgattttagtatatctttgtcgttgttttcttcattcatgtgtatttgtctgctggttaaaaaaaacagaacaaacacccataagtctgtaatttaccagcttatacgaatctggaaatgttaaaaaatgcatgttttgatgttctgcaatctgcagtcaatcaagttcatcatgatgacactggttaatggattctgcgcgaatgatttgatcttgtccatttttatgaattaaggttgtttgctgtagattgattgcagcgttctagtagataaaaaccatcatcaggtgggtttaagtccgagtttagttctatctgttcaaggtgtgagaaatggaatatttagccagaaagtgcctaagctcagagcggagataatgcacggttgttgtttccttggaggtcttagaattgatattagaccgacagtaaacgaatccaatttttcgcgtaggaattctggagtatgttattcttgtaagccttctcgtctttagcctgaaaatcttaggtttgaaggttcttccttttaagttataacccattacatcatactttgtactgcttatgttatttcagggttgtcgaatactcaagttgctagcagtgcatttacattaggaacagctgctgtcctcccattttacactctcatgatcgttgctccgaaagctgaacttgtaatcttctcagaacttactcagcaataataatgatacatcaagtttgttgatgtaacagtcgtcgttatttcttgtatgtatgaatgaatgtaaactggattactgcagactaaaaagactatgaaaagtagcataccatatgttgtgctagggcttctgtacgcatatcttttgtacctttcttggacgcctgaaaccatacgcttgatgtttgcgagtaaatactggttacctgaggttagtttgtttagcatcaactgacatattcaattatgaaatatgaaactaatttcatattcagtaatctgcatttttatggatgatatgcagcttcaaggtatagcgaaaatgttttccagtgagatgactttagcatctgcatggattcatctgctggtagtggacctctttgctgctaggtcacttcctactcaagtcaagaattatggtattctgttagaatgagacactgaattcagaagaaaaaaaaaactcacaaaatcctatatattttctgaacaggaatgtttatcaagatggtctggagaaggaagtcgagacccggcattcagtctcaatgtgcttgctattctgtcctgtaggaattctaagtcatctcatcaccacggcgctgaccagaccttctgacaaaactcgacatagcgatactattatctaatttttctgaactagagttttaatctgttttttgtgaactgatgttttggttggatgtgccaaggaagttgctgtcaaatttaaatgaaacaatgcatatagacaataattagccataagagacacttagagaaaaacattagcactgaatagttttcttgtcatgaattgatag

SEQ ID NO: 15 - DNA, 1934 bp, Valerianella locusta
  misc_feature 1..1934: note = source = /organism="Valerianella locusta" /mol_type="unassigned DNA"
  source 1..1934: mol_type = genomic DNA
cttttgccaccctcaattctcactcaaggtaatcatttaatgctttctttacttttgtttgtgtagttttatggttttttgatgttcttgattcatacccatttctcaattttgcctaattgtgaaatctttgaggagttttgattggatatgggtagttttgttgttttcttacaaagaaaatgtgaatttttggcactttattgttctgggtttgtgctagatctgagaatacttcttgttaattgttcgaatttatgcgagaatttgagtaatttggagctagtttgctttcggtttgactaatttagtgtttgatttggaaaatttggacattttaagctttaaaggtaactttctaaaccagtttatagagtcggtcaataaattcattatcggtgatgtgtcagcatcctattggataattcacactccgtatgatcagcaaaaagtgtcactgttgattgtttgatgcattgggtaattgtacattagatcagagtacaaccctttattgcatacaattagtttcagcttttgacattgaacttgtatatagaagagagttttactgtcatcaatctagttagctgtatataatccctaacattttagagcttaatttgtagatggattgctcaatatcgactgtaaaatcttcgtatattacaagaaaccaaaaacaactgacaaattttactctcgggagtacgaacggtcaaccttttggtcaacattttgcgtggaaagaagctaagctatcttgtgggtcgagtttctcaggaaggtcaaaagcaatcgtttcatcgaaccctcgaaaacttattcacttcagaaaatactgtcgaatttacgcttcatgtatatcctttcccacagaactttgaatatcaaacttttgtatgaagtttgttaaatcgtatcttttgcagggtggtcgaatcctactacaattgcgaacaatgtattcaccttgggaaccgttgccgttcttcccttctacacactaatgcttgtggctccgaaagccgaactggtaaaacctagtcgaattactctcaagtttagtacagtaatttattttttcttgctttgactaaaagattgtaatctgaatgcagacacaaaaatcgatggaaagcagcataccgtatatcgtgcttggagtattatacgcatgcttattgtatctgtcgtggtcgcctgatacattacgcctcatgtttgcgagcaaatactggcttccagaggttcgtcatttgaataaaatgctaatttggtgtttatatgttaacaagggcaaaacagtcatattttaaagtaattagattcagattagttataacccgtggtagattaacagttcttttaaattcagatagcagactttcgtaaagttttgttgagattccaaattccaaaccatcatacactatcttgcacttaaattgaccttttcggtgtttcagctgcccggtatagctaagatgttctcgaatgaaattacattggcttctgcttggcttcacttattagctatcgatctttacgctgccaggtcacctcctatctctctttctacacacacatacacataatatataccgagcctttggtattaccaacttagcgtaaaattgggtgcaaaaaaagggtatctatatgtatatatgtgtctctaatttctttatgatacacacacgcttcttttttgaacctcgaaaggcttatttgaaatacgtattatgtattcacatttaaacacattttttgcactttttggcacctgaatatcacagcactttatattttctgacattggtaatctctgttaacaggcaggtttacaaagatggaatcgagaacaacatcgagacgaggcattcagtttcgatatgtcttttattttgtccaattggaatcattgttcatta

SEQ ID NO: 16 - DNA, 1900 bp, Raphanus sativus
  misc_feature 1..1900: note = source = /organism="Raphanus sativus" /mol_type="unassigned DNA"
  source 1..1900: mol_type = genomic DNA
cccttttttagtcagtggaagactcttttaagatttcaagtcaaaaaaaaaaaaaaaaaaagactcttttaagatttgttttatttaacataaaaaatgcatttgagttcggtgtagaagctaaatgaagagccaatttccctcaaagagttcgtaaagtttgaatcggagatggctttttctcagcctctgtcttcttcgtctctcatggtatttcgcttttagttaaaaaaaaaaattattctccagtatatgtacatcagtaactaatgtatgcttatgtacagttgtttggattagattctgtgtcgagcttacttactagttagtactcacatagttcagattccttatccttaagagtcaaagttcactttccctgtctctgtctgaaaatttcagattccgtgacttaatgtcgttatcaagtttttttttttgtttgattttttttaatcagattagattctttttttttggtggtacagatgatgaatcggagctttctagctaagagctcggtgacagcaagtctttctctcaacaagtctagagtgtgcgttgattctttaaaaattcaattccagaatcattggagcttcgtcggaggatcacgactcgcttttctccctagtctttcgacgaattcatcctcctttgttcacaagaaacgctcctgcgtacgagcttcatgtaatgtctcttcttaaccggaagattttaagctttgaactttgtcgagatttaatatattatgttgatgttcagggttagctacttctcagatcgcaagcagtgtatttgcggtcggaacaaccgcggttcttcctttttacactctgatggttgtagcacctaaagctgaaattgtgagtccttttctgtgtttacaacttcttgtacagaactatgagaggttcatctgaaattgaatattatatgtgtctctctttttgtgcagaccaagaagtgtatggagagtagcataccgtatgtcgtcttaggcctattatacgcgtatttgttatacctttcttggacacctgatacgctcaaatacatgttttccagtaaatacttgttgccagaggtttgttttcaatacaaactctataacaatgttttttatatagctgctaaatgttttcttctctcttttttttttccttggtcatttgcagttgtccggaatagcgaaaatgttctcaagtgaaatgactcttgcttctgcttggatccatcttcttgttatcgatctttttgctgctaggtatgttgcaattttcaggttacttttggttttaatcaaaagttgcacatgtttcttataacagatgttttgtttgtttcttctatgaagacaagtttttaacgatggcttggagaataagatcgagactaggcactcggtttcactttgccttctcttctgtccggttggaatcgtttctcatgtggttaccaaagctttaaccaacagttctacatccaataccaataaccagtgcaagtaaactgatcatcttggttggtctctcaccattgtctttcttaactgcttataaatgtttttggtttgagatagttcattttgctttagcttcggttaagtcagcagaacgagtttgttgtggatttagttattgaaaaaaccaaataagaccaaacaacttgagacagtgtttcttttactatttggtagacataattttggattccctgatcagtcacagagattccccgtgatctctagctattttagagagtatccaactcctggaaactcaaaaaaacacacggtcacctaatttagaatactctctaacaacatttgcctgcgatctctagctatttatactatagccattataaagaactatgttttaaattgtactagctt

SEQ ID NO: 17 - DNA, 1712 bp, Capsicum baccatum
  misc_feature 1..1712: note = source = /organism="Capsicum baccatum" /mol_type="unassigned DNA"
  source 1..1712: mol_type = genomic DNA
atgaactgctggacaccagctttggtgtcaaaagtcccgctgaatacctggagaaaccagactgcctcccttgctcttagagaaatgaagtctgaccttctaagtcaacatattggtggatttgaaatcaagcatagctgtggagggagttcactggcaggatccagagtcactattcaactaaatcaccaaagaactctttctcaacgaaaaagctttagggtgtctgcttgctgtaattactttcttaaaatctccatttctttgtcataatttatctctggatttgaatgttcacgataaagtagttttaaatatgtgctttaagttattgctgcagttgggtttagtagtctcatcaatcgccttcttttttttatttggagaataaaattgcttaaaaagcgcatattttgtcattagttttaatgaattataaagcactgaagttccaatgatactgagtgtaaaataaattagagttttaacagcaatctcccttcatgcagctattaatcttccttgatccttttgtacagtttttcttattttggcagactcaatcttccttgatccttttgtacagtttttcttattttggcagactcaatcttccttgatccttttgtacagtttttcttattttggcagacttttatgccaactactaacattagctaagtgtatcactggcaagctcttagttaagtttcttattcatttatagggttgccaagttcagaagttgcatctactgctttcacagtgggaacagcggtagttcttccattttataccatcatggttgtggctcctaaagctaaacttgtaagatttctaaagtgcttttactctgaactcctttagcgatttcatttccagtgtactggagatcaaacttggcagtgaatttattaattcagaaggcgttcttaaattacacactaaccagcttcaaacaaagtagaacagttggtacacaatctcagtccttatgtatatgttttccattcagtgctttagtttgatagtatttaattataacatgctgattttggcaaaagatgtaagtcattgctttatttcaaagagcaagttgtaactgaacaaaatttcaaatgcagaccagaaaagcgatgaaaagtagcataccctacattgtgcttggacttttgtacgcatatctattatacctctcttggacaccagatacgatccggttgatgtttgcaagtcaatactggcttccagaggtctgtgctcaactacataataatttgtacaagttgtatggtcgggatcttaacacttgcttccattcagctgcctggtatagctaagatgttctccaatgaggtgacgttagcttctgcatggattcatctgttggctatcgatctttttgctgcaaggtcaatctctaggcatctatctttgttgggctatggccctttgatttctttttgggacatcatgtggagggtttcacttttagacatctaactagagtatttcacttgaaacaggcaggtttatcacgacggattgcagaatgatattgaaacacgccattctgtgtcgctgtgcttgctgttttgccctgttgggattcttactcacttcatcaccaaagctctaactagtagcccagaaaagagacagcgtaggattcattaaccaatgttttaggccagcatgtgactatcagcaaa

SEQ ID NO: 18 - DNA, 1257 bp, Chenopodium quinoa
  misc_feature 1..1257: note = source = /organism="Chenopodium quinoa" /mol_type="unassigned DNA"
  source 1..1257: mol_type = genomic DNA
atggctttttcttcctgctttgcctttcatccccagatctcttcttccaagattgattgccgagttttagtacataaaatccatcataaggcaggattaagtccaagtttagctctttctcatcagggtgtaagcactgaaatttatagccagcaagtgtctaagctaagacctgatgtaaagcatgattggtgtttccttggagggcttagaattgatgttagaccgaaagtaaacaaatttgtgttttcgcggaagaattctggagtatgctattcttgtaagatttctcttcttaatcctgaaaatgatggtttgctcaaagcctgtaacatgtgattatcagtttttatccttttcgagtttataatctcaggttcgacctttaacccaatgcagcatactttgcttgttatctcagggttgccggatcctcaaattgctaccagtgcatttaccatagggacagcagctgtcctcccgttttacactcttatggttgttgctccgaaagctgaacttgtaacttctctgaactaactgaactatgtatgaaattttttcttggtgtaacagtcatcgttaaatagtctaaatgaatgttacaccaaggaaagtgtttattgtgtgctcttctattatgtgtatgacagtatgattactgaatatactgcagacaaaaaagaccatgaaaagtagcataccatatgttgtgtttggccttctgtacgcttatcttctgtacctttcatggacacctgaaactataagcttgatgtttgccagtaaatactggttacccgaggttagtttgtttggcattaacaaattaacgacagattcaaatacaaaactaatttatattcacaattttgcattttatggatgatatgtagcttcagggtatagcgaaaatgttttccagtgagatgacattagcatcagcatggattcatctgttggtagtggacctctatgctgctaggtctcttcttccctctcctctgcttactctagtagtctagattatggtgttctattataatcaggcgttgattaaaatctaacacactcctattttgtgaacaggcaagtttatcatgatggtctacagaacgaaatcgaaacccggcattcagtctcaatgtgcttgcttttctgtccaattggaatcctaagccacttgatcacatcgtcactgaccaaacctgctgagaaaactagacatacagatactattatctaattttttctgaa

SEQ ID NO: 19 - DNA, 723 bp, Fagopyrum esculentum
  misc_feature 1..723: note = source = /organism="Fagopyrum esculentum" /mol_type="unassigned DNA"
  source 1..723: mol_type = genomic DNA
atggcgttatctacttgcttctcacatgcccggatcttcttacagaatgacatgggcagcaaggttcagaggactcagcttaacttcaggttggaaacaagacacaccgtttctcgtcaatctttgaacattcaacacttttgccaaaaccccctcagtgaacagagccttggtctaggctgcatgaccgctgctagaacaaagattaacacgacaagtctgtcaaaaaaaagacctggaatttgttcatgctggatggtagggtctcagattgctagcaacgctttcaccttaggaacggcagctgtactccccttctacacactcatggtctttgctcccaaagctgaaatgactaagaaagcaatggacagcagcataccgtatgtcatgcttggactcgtatatgcatacttactatacctttcgtggacaccagacaccataaagctaatgtttgcaagtaaatactggctacccgagttacccggtatagcaaaaatgttctcaaacgagatgacgttatcgtctgcttggattcacctgctgatagtcgacctctttgctgccaggcgtatatatcatgacggattggagaataagattgaaactcgtcattcagtgtctatgtgcttgctcgtctgccctattgggatcttgatgcatacaattaccaaagcactgaccagaacacgagttgaaagcagcaaacacaatgtatga

SEQ ID NO: 20 - DNA, 1978 bp, Lens culinaris
  misc_feature 1..1978: note = source = /organism="Lens esculenta " /mol_type="unassigned DNA"
  source 1..1978: mol_type = genomic DNA
gctgaatctgttattcactatccttgttttgcttcaaccatgtctttctcttcttgctattcccatttacctttagcatttaataaggtacactttttctgttttcatgttttttcaattctttgcacatgttgttttgtaatcttatctgcatttttcttgtctttttggtggatttttttttgtacccttttattttaatttgatttttttcaaatggggtttctgtttgaggtttaaagttttgaactttggttaaaaatatctgaaattgaaagttttttgctttctgtcattgatttgaatcaccaatgcattactaatcaaatggccatttgagttttttcttttgttgttaatttttgtatgtaatagatctgatgatgctaggtgcatgttggcatgttgatgataaactatgtagaacaacactttaggttgacggtgtgtctgatattggatgtgagtcggcggataccgatagaatactgacacacgtagttacattgaatcattctattttctcaaattatgatggtgttgacgtgtcactatcgtatctggtgttcatgttagtgtcggtgcttcgtaaaaaacaaatacgggtttgttcaaatagtccttgaatattgagctgtatgattcacctgcacaaactatgatatttcatatctgagctcaatgtagttcatttattctaattgattgatcatcactgggggcaggatataaaactctgtaggacagttggacaagagaagctgaattttcctttcactataaggagtaatagtgttgagctgtgcacccgacgcatttcgagcagtagagccggcttaagtggagattggagtttcataggaggatccaaaattgtagtaaaacctaaagctacaacatcgtttcgcaatccaaaacgaagtcaaatacatgcttcatgtaataatctcttttcatgctacttaatggtagggataatggtgacaatatttgttctgcatgttcattgttctagctctatgtttcagggttcataggatctcaacttgctagcactgtgtttacatggggaacaatcgcggtgctcccgtattacacacttatggttttcgccccgaaatccgagctagtacgtttgattagtgattgcaattcacttcattaaaataacatattgatattcttgtttttcatttcatttatttggttatgattctgatatcctgattcatttttctgaaatgcaaaattacagaccaaaaaggctatgcagagtaatttaccgtatgtaatcctcggcgttctatacgcttacttactgtgcctttcttggacacctgaaacggttcgattgatttttgcaagtaaatacttactacctgaggtgagtagtcattcattcatcgatgaagttcagttttctttctctaatgagttcttttatctaactcgtaactgtttatattcgctactccatcatgcagcttagcagcataggaaaaatgttctctagtgagttgactttagcctctgcttggattcaccttttggttgttgatctttttgctgcaaggtccggcattttatcttcctttttgcgataagatttgatatttggacacaaaaatcagcaacaatttggataaacatcgttcaaatatatggttaatcgcattcagtgaatggtcaatgaatacaactctaaattaatcatgtatttgagtcgcattaactctaaattgttgtcgaattttgtgtcaaaataacaactatttctcattctttagctatttttctaatagtatatttggttcaaaatccaggcatattttccgcgaaggaatggagaatcagattgaaactcggcattcggtttccttttgcttgttcttttgccctatagggattcttactcatgtcatcactaaagcaatgaccaaaactacaagaaaacagggtcatggtttatagatggcac

SEQ ID NO: 21 - DNA, 3149 bp, Medicago sativa
  misc_feature 1..3149: note = source = /organism="Medicago sativa" /mol_type="unassigned DNA"
  source 1..3149: mol_type = genomic DNA
atcatgtctttctcttcttgctattctcattcaccattaccatttaataaggtacamccctttcattgttttgttttgtaatcttatctgcattttttttgtcttttttggtacctttttttgattttacacaaatggggtttctgtttgaaatgtaaagttttgaactttgaataaatgtatctgaaattgaaaattgttttctgtgatagatcaraatcaccaatgcrttaywaatgtgaaawgggkctttgagttttttttttttttttgttatttttaagtttgtaatagatttgatgttaggtgcatgttggtattaaatatgtagaattgacacttcacattgatgtcagtgtcatgtttgtgtaagtgcttcataggcaataaaagggagtttatattgccgcgtaagtataactcagatggtaaaatgttgcagtgacatttgatatgttaaaatgcatgttggtatattgtcgcgtgagtacacctcatatgatagaatgttgcagagaaatttgatatgttgtggcgtcggttcaacccctcattttcaacttcttagcacttggttggtgtgagttttgccgctaggttgtttaaaacaaaacaaataggagtttgtatttcaaaaagttggcactcttgtgtcatcaaaccaactttggagcaccgacacttaaaattgaagatttgtccagtgtttagcatgtgtcgatgtccaacaccggcatatgcggttacattgaattatttcattttttgagtcaatgtagtttatttattcgtatgtatggataatctagtgtgtatttctgagctcaagaagttttattctatttcatattgatttataatcatttggggcaggatataaaactctgtaggacagttgggcaactgaagctgaattttcctttctctatcaggagtgatggtgttaccaaacacatttcgagaagtagattcagtttaagtggagattggagtttcataggagggtccagaattgttgtaaaaccaaaagctacaagatcggttcgccatccaaaaagaagtcaaatacatgcttcatgtaatccttttttaatgctactttttcatgtaatctagaattggtgcaatttgtttcttacatataatttaccattcaatagaattggctgtgaaggaatttragcataatggatatatttaggttcttttgcaaaaattgttggatctgtaaggatctgatacacaagatgcatctctatatttatcttatcttttttggcggcattatcataaagtaggttactattagggcatgtttggattgacttatttgagcttatctattgatatagagcctagtaagactgtttgagacttgagagaggttatgaaaacacttatacatgacatgtgcataagctgtttttagtttatttccttaaatgctttaagatagtttattgaaacagcttatagattatatgaaaacagtccaactttattttattgtttgttataaaaatagcttagacagaagcacttatatgataagcgtcagctaagctgtttatccaaacagggtcttgtcttttctgagctctattctttttaagtttttggagacaagttatggatgttaacattgctccttttgcatgtattcccttttctacaattattcatgtggcccctgatctcagctattcgagtttcctaattttctgttattcttttgtatattgtaactttcaaagccttgaacaaacacatttaggtcgacaccattgaatcgaatarattgttataatatacttgaaaaaacttgattatgatctatgcttaaattgcttgttctgtataaatggyggtgattcattgttttacctcaatgttgcagggttcataggatctcaacttcctagcactgtatttacatggggaacaattgcagtgctcccgttttacacccttatggttctagccccaaaatccgatctggtacgtttctttctgcatttgagaaaaattatgattagtaatctcattttcacaattcatattcagtttttaggtacattaacaaaaaagcattctgatattccttttcatttcatttatttggttatgatactgatatcctgattaatttttctgaaattaaaaaatatagaccaaaaagtctatggaaagtagtttaccatatgtagtgctcggcattctatatgcttatttgctgtgcctttcttggacacctgaaacagttcgattgattttcgcgagtaaatacttactacctgaggtgtgtattcattcatcaacgaagttatgttttctttctttaaagagttctattattcaaactcataaccgtttatatttgcatactccttgcagctttctagcataggaaaaatgttctctagtgagttgactttagcctctgcttggattcaccttttggttgttgatctttttgctgcaaggtcctgttgtatcttttgtgatttctacttcacccaattttcctcgttattgctggtttttcattcatgaatgatattttgatacaaatttgcgaacaaaaaatcgagaacaatttggataattaatgccgttaaggtayctggttgatcgwattaakkggttggttaatgaatataaktatatgtcacaactcattaatcatccggttaatgcaattaaccctgaatttggacgtcataaaccaatggtttttagatgttcaaatatacatggtatccattaatcatcccaattatattcatgatcttcaggttttcgaatgcacatgatattctattaaccataatctgttaatctgtgttaaactatacacatgatatcgtggttaatatcgtgattaatgacattcaaaaccgtggtgaattttgttgtcgaatttgtgttaaaataacacagctctttctcattctttagttatttctctgacagtatttttggttcaaaatccaggcatatatttcatgatggactgaagaatcagattgaaactcggcattcagtttccttttgcttgttcttttgcccaattgggattcttactcatgtcatcaccaaagcaatgaccaaaactacaagaaaagatggtcatggtttatagatggcac

SEQ ID NO: 22 - DNA, 393 bp, Pisum sativum
  misc_feature 1..393: note = source = /organism="Pisum sativum" /mol_type="unassigned DNA"
  source 1..393: mol_type = genomic DNA
atggttttcgccccgaaatccgaactaaccaaaaagtctatggaaagttatttaccgtatgtaatcctcggcgttctatacgcctacttgttgttcctttcttggacacctgaaacggttcgattgattttcgcgagtaaatacttactacctgagcttagtagcatagggaaaatgttctctagtgagttgactttagcctctgcttggattcatcttttggttgttgatctttttgctgcaaggcacattttccgcgatggaatggagaatcagattgaaactcgacattcggtttccttttgcttgttcttctgccctattgggattcttactcatgtcatcaccaaagcaatgactaaaactacaagaacagagagtcatggtttatag

SEQ ID NO: 23 - DNA, 2958 bp, Vigna radiata
  misc_feature 1..2958: note = source = /organism="Vigna radiata" /mol_type="unassigned DNA"
  source 1..2958: mol_type = genomic DNA
tgaatcacttattagctcttttgcttttccttcaatcatgtctttctcttcttgcctttcccattccccattgacactcaaggtacactttctcttagctttcctattgctgccattgatttctaattttacatgcaatttttcttccacctttttgctcattcgctaccttttatttatcacttattttctttcctggcttcagctcatttcccccatgcccactagattggagtttgattccctacgtttgaactctaaagttttaaactttgaatggttattggaccgaaagtggccattttgcgtagatttcaaccacctaagcattaccaacgaattgggcatttgtgaatttatttttttgctttgcatggttgtttgcttgttttgctttgcatggatctattctaggcgcttgttggtgtagtagagttaaaaaggagtttgtatttctgaactggcttttccgtgtcttcaaaagctctaaattcattcagttctgtgggtttgttcaaagagtccttgcgtgttgaagtttcattcaaataataatctgcacaacctggttatttccactctagaaaaggtttaatataatttattcgtatatatggatagcataaggtgtactttctgggcttaagacaaactgtgcttataattgagattctgtttgtttcattttggcagcctataaaaccttgtggttctgttgggatgaggcaaaattttgctttctctttcagaagtaattggcctgagctttgtaacagacacattgtagggagtagaaggttgcagggaaatttaccaagggtcaacttaagtggagattggagtttyataggaggatccaaaattgttatgaaaccaaatgctacaagattgcttcattatccaaaaaggggtcaaatgcaagcttcatgtaaccctcttatactacagcttctcattttcaaactcattttgaaaataacgtgtgtcttgtgctggaccaaatttatttaagaaccaattgaagtctctggtatttttgatgtggtgatacttttctgtgtctctgagcaacttacaggtgaaattggaggttttataattaggcctctttcctctaaatttttctcattttgaccaccctggaaaatttcactgcattctgatttatataaatatcattagcgcaagctgtttcttcattcatatattttgattcttattaaaaaactgttggatttgtcttgccactaaactaatttgtttatctcgaaatagagcacaaattaaggatttgattcacagaatgaatttacatggttagcttaaattacccctcgtgtcagtatatctataacttaaattactgtatgatatacacgcacattgaaactaccgagagctataaatatccgtgcattgtctgcatgacttcaccaagtgttgttcttagttcaagcttaaccaagttactccgctttattttttgaaatttttagggaccagttattgattttaagttgtcccttttgatttagtcttccccattttcatgtggctgccgattccggctatctgtgctgttgtggttcctactttttcattattctctagcataatgtgactttgaatttgatagccttgaggaaagtcattttgtttggacagaaaactctttaatgtcgaatctgaacagctttttctaacatggtgcttaaaatttaaatcttgctactagttctgctcttgaagcagatgttcaatttcttggaaaggtatgctaggaatcaggtttcactgaagctattcagctgtggtctaaatttcgtacgaccattacattcattatggttgggtttaaagtctgcctttacctttcgatatttttctattttactgttaaagcaatcgatcacaatgagtaattctaaatagcaaagatgtgcttattgttatcttaactacttagacattttggtaatctgtttctctttgtataaagttgactgaatgttcctttattctgtataactgatggtgactatatttttcgcctgatactcacttttcttcctttcattttcaggcttcataggatctcaacttgctagcactgcatttacggctggaactgtagctgttctcccattttacacacttatggttctagctccaaattctgatctagtatgtttctaactgcagtggagaaaatttacgaccaacgagcacgattcattgcaacaactttgctttattacatgtctgtttagttaccatgcaaaaatcattcacatatataattattttctatagtagtaaataatccttgtgtggaatttggatattcttctttctcgtaagcttctattgggtctctgattttgtacttcacgtctttcctgattcatgttaagtgcaaaaatgcagaccaagaagtctatggagagtagtctgccatatgtagtgcttgggattctttatgcatatttgttgtacctttcttggacacctgagacagttcgattgatttttgcaagtaaatacttgctaccagaggtgtgtgtgaatgcattcagcaatgaagtttttcttcccaaaagagttgtatgcaactgataaatctgaatacttgatgcagctgcctggtatagcaagaatgttctccagtgagttgactttggcctctgcatggattcacctgttggttgttgatctttttgctgcaaggtcgtggattttatctttctcttggtttctcattctttacttatttatctaatcctatttctggttatgaattcaggcatgtttttcaagatggactgaagaatcagattgaaactcggcattctgtttctttttgcttgttcttttgccccattgggattcttactcatatcatcaccaaagccatcaccaaagctgccacaaaagagggtcatggtttatagatggcac

SEQ ID NO: 24 - DNA, 744 bp, Vigna radiata
  misc_feature 1..744: note = source = /organism="Vigna radiata" /mol_type="unassigned DNA"
  source 1..744: mol_type = genomic DNA
atggctttctcttccttctttttccattctccgacactattgaagattgatcacttggggcagactaaaagaccttgtggtaaagttgaaaaggggcaaaagtttcctttctctgtcaggagtaatggtgctgagactgaactttgtaaccagagtcaacttagtcagagaagtagagtcagagattggagtttcatgagaggatcaagagttgctatgaaaccaaaaatcttgagattggctccttctcgaaaagtccctcgtctatatgcttcatggttgtcaggatcagaacttgctagcactgcctttacattaggaacaaccgcagtgcttccattttacacactaatggttctagctccaaattctcaactaacgaagaagtctatggaaagtagtgtaccatatattgggcttggagttctatatgcatatttattgcacctttcttggacccctgagacagttggacttatttttgcaagcaaatatttgctaccagagctgactagtatagggaaaatgttctccagtgagatgactttagcctcagcatggattcaccttttggttattgatctctatgctgcaagacatgtttttctggatggacttgagaatcagattgagacaagacattcagtttctctgtgcttgttcttttgccctattggtgttcttactcatgtcatcaccaaagcaacgactaaaagtagcagagaaaacaagagtggattatag

SEQ ID NO: 25 - DNA, 3249 bp, Trigonella foenum-graecum
  misc_feature 1..3249: note = source = /organism="Trigonella foenum-graecum" /mol_type="unassigned DNA"
  source 1..3249: mol_type = genomic DNA
tgtctttctcttcwtgctattcwcaytcrccattgccatttaataataaggtacaacactttctctgctttcttttcctgttttttcaattttctgttttgtaatcttatctgcatttttcttgtcttttttatggatattttgtacttttttttttttttaattttccacaaatggggtttctgtttgatgtgtaaagttttgaactttgaataaatatagctgaaattgaagattcttttttgtcatagatttgaatcaccaatgcattactaatgaaatgggcctttgagcttttattttttagtttgtaatagatctgatgctaggtgcatgttgatgttggtatattggtaatgaactatgtagaagctacacttcagattgataatgtgtctggtgtttgacacgtgtttgcggatacaacacgacattaacacatgtggttgcatttgatcactttcattttcttaaattgttacaggtgtctacgacttagtgtcgtgtcgtgtatgtgttagtgtttcaaaaagttgacactcctgtatmaacaaaccaatatgtgtaaaaaaaactatgtagcaccgacacttcatattgaagatatgtatggtgtttgagatgcatcagtgtccagcaccgacacaatactgacacatgtggttacatttaattayttcattttctcaaattatgatcaatgtcaatctgtcagtgtcgtgtctggtgtccgtatctggcttcattggcaacaamtatgtatttgttcatgtagtcattgcatattgagktgtaagaatcgtcagcrcgacctgtatatttcctgttgaagatcaaacaatttagttcatttactcttaygaatggataacctagggtgtatttctgggttcaagaaattttattctattattgattgatcatcacttggggcaggatataaaactctgtaggacagttgggcaagtgaagttgaattttcctttcgctataaggagtaatggtgttgagctgtgtactcggcgcatttcgagatgtagattcgacttaagtggagattggagtttcataggagggtccagaattgttgtaaaacctaaagctgcaagatcggttcgctatacaaaaagaagtcaaatacatgcttcatgtaatcttttttcatctaatctaaaatttgtacaagctgttccttagttcatataatttaccattcaktagaattggctgtgasggcgtttgaacataawaaagttaaattgytttcwtataacctataagtttttttcstawsttatattckagagcttacraaaataarctgaaaacaacttatggacatgtcgtaacctgtttccagaaactatactaaacagtctcataasttcttatgccaataaataagctcaaataastcaatccaaacaggaatgcatttaatttttargttaccatttttggtggcgttatcataaagtagattactgtaagtacttttgtcttatcatctttatatgaacaacgaaactggaggcagtggttaatatctgttcattgatcatggtgtacaatgctatatatgataarttataaccttgcaatgtgttgctgaaggcaatatggttcacaattcatgctttagttgagttagggtctgtttggattckcttatttgagtttaccttctaacataagcatttgtgagactgtttgagagagtttatggaaacaacttatatacgacatgtgcataacttgttttaagttaatttttataaattctccaagatagcttatgaaaacaacttacagattatatgaaaacagctcgactttattttattttttgttatagaaataacatatgcataagcacttatatgataaacaaggttttcttgtttaggtggataccattgacttgaattgcttgttmtaatatacytgaaaattgaytaygatctatgcttaaattgcttgttctgcatattcaytgtggttcatgggatctcaacttgctagcactgtatttacatggggaacgattgcagtgctcccgttttacacccttatggttctagccccgaaatccgagctggtacgtttcttttttgtatttgtgaaaaattatgattagtaatctcatttcacaattcatattcagttatgatattctttttcatttcatttatttggttatgattctgatatgctgattcggttttctgaaatgcaaaaatacagaccaaaaagtctatggaaagtaatttaccatatgtagtgctcggcgttctatacgcttatttgttgtgcctttcttggacccctgaaacagttcgattgattttcgcgagtaaatacttactacctgaggtgtgtattcatttattaatgaagttaaattttctttctctaaagagttcaattatcaataattgtgttatatttgcatactctatgcagcttactagcatagggaaaatgttctctagtgagttgactttagcctctgcttggattcaccttttggttgttgatctttttgctgcaaggtcctgattttatctctttgtttttgttgctcagtaatgagattttgacacaaatttgacaaaaaaaagtagaaaacaatttggatagttaatgccgttcgaatatgcggttaattacatagtgaatggttaatgaatattacaaaatacaaaatgtcacaagtcattaaccctgattttgaacgccgttaatcataaactttaggtgttcaaacatacgtgatattcattaaccattccaattatgttcacgatcttcaggttttcaaatatacataatattctattaatcacaatttttgttcaaatatacaaatgtaattgtggttaatgacattcaaaatagtggttaattgtgatctattgatgggtaatgagttatgacactttgttataatcagtaaccatctactaaatgtaattaaccttatatttgaactacattaacatttaaattgttgtcaaattttatggtctaattttgtgtcaaaataacacggctctttctcatgcttaaattatttttctgatagtatttgtggttctaaatccaggcatattttccgcgatggaatggagaatcaaattgaaacacgacattcggtttccttttgcttgttcttttgccctgttgggattgtaactcatgtcatcaccaaagcaatgaccataaaaacaagaaaagagggtcatggtt

SEQ ID NO: 26 - DNA, 1845 bp, Cichorium intybus
  misc_feature 1..1845: note = source = /organism="Cichorium intybus" /mol_type="unassigned DNA"
  source 1..1845: mol_type = genomic DNA
atggctttctcttcttgtctttgccaccatcaattggcactcaaggtattggttaatttccctttttactctctctatgtgtgtttgcatatgctcaaacgacttcactttcacgaattcatggtttatttggcattttgcgatttgggtacgagtcatttcgcgttattggtactaaatctggttgattttgccgatttaactaccagtgtcatccaatttgtgcattttcacatgtttttagctacctcacttttacatattcctgtttgtttgcgaatttactatctgggtgtgattcagtttgctgtgttcgtgttaatttggttgttttggctcatttgattctgtttattacatccatttctgtattgtgtgactgcagattgaatcattcactttacatatacatattatgctgtctgtaaatctattcgtttgtatcttctccccaattgaattggttcacttttccgattttgatttcggttagcagtttagggttcatagatgtttatgttcaaattagaaccatcaaaagggttacattagtgagaaatcttgaagatgttaaatctttgttgcagatcaacctcttaacgagtccatcaaaacccacattcgctcttaaagccatgaacaccgaattttacggaatacatatcggaagcaagctaggaaatcaatggagttttatgaaaggatcacaagccataatcagaccgaaccctggaagcttcaatctgcatcaaaaaagctcaaaattgcaagcatcatgtaatcctttcgtaccctttgtttatcatgatacaatttatcgattaaacatccaaaactttgttaatcttatcgttttttagttcgattggatattttttcatgtagggtttgcgagtatgcatttagcgagcgatgcttttacattaggaaccgctgctgttcttccattctacacccttatggtcgcagctccaaaatccgaattggtaaggtttataatgttgtcataaagcaaagaaaattaaaaaaaaaacaaaaaaaaaaaaaaaattcattcaaatacctatatcaatatagttggaatttaagtgatgtttctttttgactcatttaaagtgttgaatggataaattgttttttttttcttttttgggtaaagtgtcgaacatggtatatattaattgtttaatatattaagttcattaagtaaaaaagaagctaattgtttacaaatttggttgacattaatgcagacgaaaaagtgtatgagaagtagcataccgtatgtggtactcggggttttatactcgtatcttctttacctctcgtggacgcccgacacagtccgattaatgtttgcaagcaaatactggctgcccgaagtatgattttacacccctatagtttgctagatagccgacttttaaccctagtgatggttttatttgcagcttccgggtgttgctaagatgttttctaatgagatgacattagcctccgcttggatccatttgttagccgtcgacctctatgctgcaaggtaggagggcatttacgtcttttacacaaacaacatatcgaaagctagtccatgtcccaccttcttccgtaggatgaaaaattgcaatttttttcccctgtacctgtacctgtacctgtacctgatgaattgtggttttgattggtggaaacagacaggtgtatcatgatggattggagaaggagatcgagacacgacattcggtttctctttgtttgttgttttgtccgattgggatacttgttcatgccatcaccaaggctttgattagtacatatagagaatcaaaaacagagattcattga

SEQ ID NO: 27 - DNA, 687 bp, Allium cepa
  misc_feature 1..687: note = source = /organism="Allium cepa" /mol_type="unassigned DNA"
  source 1..687: mol_type = genomic DNA
atgcctctcctttgctcctgcgattccaggatctataaacaggcaactccattgtcaaatcaactgaataaatggcgaggtcttagttcacatgcccaacaattcattcctaatggaagcaaagatatagttcaatggagttttaaaggagggtcaaagatagttattcaaccaaaaatatcaaagatcagttaccacaaaagaggctccgacatatctgcttattggattcctacatcgcaaatagcttcgaatgccttcacaatgggaaccgttgccgttcttccattttatacgttgatggttgttgctcccaactcaaagcttacaaaaaggacaatggaaagcagcataccgtatgttgttcttggtatgctatacatgtatcttctatatctatcgtggacacctgagacgttggggtatatatttgcaactaaatattggctgcccgagttatccggcatatcaaaaatgttctcaaatgaaacttgcacgtcttctgcctggattcatctactgactgtagatctttttgccgcaagacaagtattccaagatggtataaagaacaagatagaaacccgacattctgtttcattgtgccttctctgttgtccaattggtatcgccactcacgcaattacaaaagctctgaagagggtgtcagatagtcgatcacactga

SEQ ID NO: 28 - DNA, 750 bp, Allium cepa
  misc_feature 1..750: note = source = /organism="Allium cepa" /mol_type="unassigned DNA"
  source 1..750: mol_type = genomic DNA
atgtctctccattacagcttttgcaacacccgcatctctcatcaggttgttcattcatggaatgctccagatagatatgcagtttatgcatttttatcagctagaaataaacatgatgaacatattgggcgacaggtagcacatacaaaaagcagaaacagggttaaatggagcttcagaggaggatcagagctgtttattcaaccaaaagccacaaggactgaccgtcaaaaacatcgatctgctctgttaacatcgtgcttaacaagttcacaaattgctgcaaaagcttttacatggggaaccattgcagttcttccattctacacactaatggtagtagctcccaatgctaaacttactaaaagagccatagaaagcaacacaccatacatcattcttggagcaatatacagctaccttctctacctgtcctggagtccttccacattgcgaacaatgttcgctagtaaatactggttgcctcagttatctggcatctgcagcatgttctcgaaggaaatgaccgttgcttcagcttggattcacttgctagctgtggatctcttcgctgccagacaagtatactgtgatggcatattgaacaacatagaaacaaggcattctatttcattgtgccttctcttctgcccaatcgggattgcgattcatgccattaccaaggcacttaccaaatattttttgaactataatttttcggaagagatgaaactggggctaaggagttag

SEQ ID NO: 29 - DNA, 747 bp, Hordeum vulgare
  misc_feature 1..747: note = source = /organism="Hordeum vulgare" /mol_type="unassigned DNA"
  source 1..747: mol_type = genomic DNA
atggccgcccctcttccctccccccttccccgagcccggcagctccaccacctcgtcgactcccggcaagaaatggcggcctcccccaccgccctcgccctcgccctctcccccaccacgcgggtggttgtcaggcggacgccggcgccgcgcgtggccgccgtctcccccggccagctccgcgcgagctcctggggcgcgccgctccctctccggccggagctcgccgcggcccctcctcgacccggcgccgcccgccgcagggcgcctctgctccggcctcgagcatggctgtcgacgtcccagatcgccagctccgccttcaccctgggcaccgtcgccgtgctccccttctacacgctcatgatcgccgcccccaacgccaacatcactaagcgcacagtggagagcaccgccccctacgtggccctcggcatcctctacgcctacttgctctacctctcctggacccccgacaccatccgcgccatgttcgccagcaagtactggctcccggagttgcctggcattgtgaggatgtttgcgagcgagatgaccgtcgcctccgcctggatccacctccttgccgtcgacctcttcgccgcaagacaggtgtaccatgatggcatcaagaacaacatcgagaccaggcattcggtttccctgtgcctgctcttctgccccatcgggatcgccgctcacgcgctcactaaggtactggcggggtcgacagggcgatcgcactga

SEQ ID NO: 30 - protein, 283 aa, Daucus carota
MNKFVLENQNALLVSILKLGQYLPSWTWELLKYLSLYCLPNAYDENLETECLTEHSSLTRKGFYNISKIQLNPVAIEGTNSDLYGQHVVLWTKMRKEWSFKRGSISIAGPTMERFVLHRKSSGVQASWFTNSQIASSVFTLATAAVLPFYTLMVLAPKATLTKKCIQSAVPYVGLGLLYAYLLYLSWTPDTFRLMFASQYWLPELSGIAKMFSSELTLASAWIHLLAVDLFAARQIFQDGLQNSVETRHSVSFCLLFCPIGILSHEITKALTTGGRTAKREIH

SEQ ID NO: 31 - protein, 261 aa, Daucus carota
MASLSCLCSSPLFLKNDESRLANKSLLAYTRKDRITTYCLNSVETDPFSRHPHSIKTKRWSFKGGSRVITGPNIQRFACYRKSCGVYALWLTNPQIASSAFTLGTAAVLPYYTLMVVAPKSELTKKSIESGIPYVALGLLYGYLLYLSWTPDTMKMMFASEYWLPELSGIAKMFSSEMTLASAWIHLLAVDLFAARQVYQDGLENKIETRHSISLCLLFCPIGIISHVVTKALTKSTEFPGFAFHNFSRLFHDILLTIANF

SEQ ID NO: 32 - protein, 234 aa, Cichorium endivia
MAFSSCLCHHQLALKINLLTSPSKPTFVLKAMNTEFYGIHIGSKIENQWSFMKGSRAIIRPNPGSFNLHQKSSKLQASWFASMHLASDAFTLGTAAVLPFYTLMVAAPKSELTKKCMRSSIPYVVLGVLYSYLLYLSWTPDTIRLMFASKYWLPELPGVAKMFSNEMTLASAWIHLLAVDLYAARQVYHDGLEKEIETRHSVSLCLLFCPIGILVHAITKALISTYRESKTEIH

SEQ ID NO: 33 - protein, 226 aa, Solanum melongena
MNCWAPASVSLSTRRNHTAFLALREIISQRIGGFGTKLSSGGSSLGGSRVIIQLNLQRTLSQRKSSRVHACWLPSSEIASTAFTVGTAAVLPFYTVMVVAPKAELTRKAMKSSIPYIVLGLLYAYLLYLSWTPDTIRLMFASKYWLPELSGIAKMFSNEVTLASAWIHLLAIDLFAARQVYHDGLQNDIETRHSVTLCLLFCPVGILTHCITKALTSSPEKKQHRT

SEQ ID NO: 34 - protein, 249 aa, Solanum melongena
MALSSTCFCHSQFSLKMESWTPALSSNIRCYIRRNQFPSSMLKTINSDLSSQQVQERGTKHSNGSSFLGGSRVMRQPNLQNLPQRRSCRVSAMWLPSSQVASSVFTLGTAAVLPFYTLMVAAPKAELTRKLMGSAIPYVALGLLYTYLLYLSWTPDTIRLMFASKYWLPELSSIAKMFSSEMTLASAWIHLLAVDLFAARQVYHDGLQNGIETRHSVSLCLLFCPIGIVIHLLTKAVLSNAENIVPRTH

SEQ ID NO: 35 - protein, 246 aa, Solanum lycopersicum
MYFSSSSHVSLKMNCWAPALASKVPLNTRRNQTASPALRQMKSDLLSQRIGGFGTNLSSGGSSLGGSRIITQLNLQRTLSRRKSPMVSACWVPSSEVASTAFTVGTAAVLPFYTVMVVAPKAELTRKAMKSSIPYIVLGLLYAYLLYLSWTPDTIRLMFASKYWLPELSGIAKMFSNEVTLASAWIHLLAIDLFAARQVYHDGLQNDIETRHSVSLCLLFCPVGILTHCITKALTSSPEKKQHRTH

SEQ ID NO: 36 - protein, 250 aa, Solanum lycopersicum
MALSSTCFSHSQFSLKMDCWTPALSSNILCYIRRKQPPSSTLKTINSNLLSQQVHKRRTKHGNGWSFLGGSRVKCQPNLQNLPQRRSYRVSAMWLPSSQVASSVFTLGTAGVLPFYTVMIAAPKAELTRKLMDSAIPYIVLGLLYAYLLYLSWTPDTIRLMFASKYWLPELSGIAKMFSSEMTLASAWIHLLAVDLFAARQVYHDGLQNGIETRHSVSLCLLFCPIGIVIHLLTKAVLLSSAEKTVFRTN

SEQ ID NO: 37 - protein, 234 aa, Capsicum annuum
MNCWTPAFVSKVPLNTWRNQTASLALREMKSDLLSQHIGGFETKHSSGGSSLAGSRVTIQLNHQRTLSQRKSFRASACWLPSSEVASTAFTVGTAVVLPFYTIMVVAPKAKLTKKAMKSSIPYIVLGLLYAYLLYLSWTPDTIRLMFASQYWLPELPGIAKMFSNEVTLASAWIHLLAIDLFAARQVYHDGLQNDIETRHSVSLCLLFCPVGILTHFITKALTSSPEKRQRRIH

SEQ ID NO: 38 - protein, 232 aa, Brassica oleracea
MAFSQPLSSSSLSMTNRSFVAKSSVTASLSLNKSLKIRFHNRWSFDGGSRIVLFPSVSSDSSSLVHKKRSCVRASWMATSQIASSVFAVGTTAVLPFYTLMVVAPKAEITKKCMESSIPYVVLGVLYAYLLYLSWTPETLKYMFSSKYLLPELSGIAKMFSSEMTLASAWIHLLVIDLFAARQVFNDGLENKIETRHSVSLCLLFCPVGIVSHVVTKALTNSSTSNTNNQCK

SEQ ID NO: 39 - protein, 247 aa, Apium graveolens
MPLSSCLYCYQISSLKTEHSTLSTKPLCNIGQSRLNTVAIEGINSDLYGQHLVLWTKMRKEWSFKGGSTSIAVPTIQRSVLYRKSLEVQASWFTNSHIASSVFTLATAAVLPFYTLMVLAPKANLTKKCIQSTLPYVVLGILYAYLLYLSWTPDTFRLMFASQYWLPELSGIAKMFSSELTLASAWIHLLAVDLFAARQIFIDGLQNYVETRHSVSFCLLFCPIGILSHEITKALTTGGRNTKRQIR

SEQ ID NO: 40 - protein, 241 aa, Apium graveolens
MASFSCLCSSSLFVKNDDLRLTNRLLEACFRKDQLTTCALKSFKTDPFSRHPPSIKTKSRTEWSFKGGSRAIPGPTIHKFARNRKSCGVYASWFTNPQIASGAFTLGTAAVLPYYTLMVVAPKSELTKKSIESGIPYVTLGLLYGYLLYLSWTPDTMRLMFASQYWLPELSGIAKMFSSEMTLASAWIHLLAVDLFAARQVYHDGLENKVETRHSISLCLLFCPIGIISHVVTKALTKSSK

SEQ ID NO: 41 - protein, 250 aa, Spinacia oleracea
MALSSCFAYHPQISSKIDCSVLVDKNHHQVGLSPSLVLSVQGVRNGIFSQKVPKLRAEIMHGCCFLGGLRIDIRPTVNESNFSRRNSGVCYSWLSNTQVASSAFTLGTAAVLPFYTLMIVAPKAELTKKTMKSSIPYVVLGLLYAYLLYLSWTPETIRLMFASKYWLPELQGIAKMFSSEMTLASAWIHLLVVDLFAARNVYQDGLEKEVETRHSVSMCLLFCPVGILSHLITTALTRPSDKTRHSDTII

SEQ ID NO: 42 - protein, 239 aa, Valerianella locusta
MAFSSCFCHPQFSLKMDCSISTVKSSYITRNQKQLTNFTLGSTNGQPFGQHFAWKEAKLSCGSSFSGRSKAIVSSNPRKLIHFRKYCRIYASWWSNPTTIANNVFTLGTVAVLPFYTLMLVAPKAELTQKSMESSIPYIVLGVLYACLLYLSWSPDTLRLMFASKYWLPELPGIAKMFSNEITLASAWLHLLAIDLYAARQVYKDGIENNIETRHSVSICLLFCPIGIIVHYITKALTI

SEQ ID NO: 43 - protein, 225 aa, Raphanus sativus
MMNRSIIANSSVRASLCLNKSRVCVDSLKIQFQNRWSFIGGSRLAFLPSLSSNPSSFVHKKPSCVRASWLATSQIASSVFAVGTTAVLPFYTLMVVAPKAEITKKCMESSIPYVVLGLLYAYLLYLSWTPDTLKYMFSSKYLLPELSGIAKMFSSEMTLASAWIHLLVIDLFAARQVFNDGLENKIETRHSVSLCLLFCPVGIVSHVVTKALTNSSTSNTNNQCK

SEQ ID NO: 44 - protein, 234 aa, Capsicum baccatum
MNCWTPALVSKVPLNTWRNQTASLALREMKSDLLSQHIGGFEIKHSCGGSSLAGSRVTIQLNHQRTLSQRKSFRVSACWLPSSEVASTAFTVGTAVVLPFYTIMVVAPKAKLTRKAMKSSIPYIVLGLLYAYLLYLSWTPDTIRLMFASQYWLPELPGIAKMFSNEVTLASAWIHLLAIDLFAARQVYHDGLQNDIETRHSVSLCLLFCPVGILTHFITKALTSSPEKRQRRIH

SEQ ID NO: 45 - protein, 266 aa, Chenopodium quinoa
MAFSSCFAFHPQISSSKIDCRVLVHKIHHKAGLSPSLALSHQGVSTEIYSQQVSKLRPDVKHDWCFLGGLRIDVRPKVNKFVFSRKNSGVCYSCSTFNPMQHTLLVISGLPDPQIATSAFTIGTAAVLPFYTLMVVAPKAELTKKTMKSSIPYVVFGLLYAYLLYLSWTPETISLMFASKYWLPELQGIAKMFSSEMTLASAWIHLLVVDLYAARQVYHDGLQNEIETRHSVSMCLLFCPIGILSHLITSSLTKPAEKTRHTDTII

SEQ ID NO: 46 - protein, 240 aa, Fagopyrum esculentum
MALSTCFSHARIFLQNDMGSKVQRTQLNFRLETRHTVSRQSLNIQHFCQNPLSEQSLGLGCMTAARTKINTTSLSKKRPGICSCWMVGSQIASNAFTLGTAAVLPFYTLMVFAPKAEMTKKAMDSSIPYVMLGLVYAYLLYLSWTPDTIKLMFASKYWLPELPGIAKMFSNEMTLSSAWIHLLIVDLFAARRIYHDGLENKIETRHSVSMCLLVCPIGILMHTITKALTRTRVESSKHNV

SEQ ID NO: 47 - protein, 242 aa, Lens culinaris
MSFSSCYSHLPLAFNKDIKLCRTVGQEKLNFPFTIRSNSVELCTRRISSSRAGLSGDWSFIGGSKIVVKPKATTSFRNPKRSQIHASWFIGSQLASTVFTWGTIAVLPYYTLMVFAPKSELTKKAMQSNLPYVILGVLYAYLLCLSWTPETVRLIFASKYLLPELSSIGKMFSSELTLASAWIHLLVVDLFAARHIFREGMENQIETRHSVSFCLFFCPIGILTHVITKAMTKTTRKQGHGL

SEQ ID NO: 48 - protein, 239 aa, Medicago sativa
MSFSSCYSHSPLPFNKDIKLCRTVGQLKLNFPFSIRSDGVTKHISRSRFSLSGDWSFIGGSRIVVKPKATRSVRHPKRSQIHASWFIGSQLPSTVFTWGTIAVLPFYTLMVLAPKSDLTKKSMESSLPYVVLGILYAYLLCLSWTPETVRLIFASKYLLPELSSIGKMFSSELTLASAWIHLLVVDLFAARHIFHDGLKNQIETRHSVSFCLFFCPIGILTHVITKAMTKTTRKDGHGL

SEQ ID NO: 49 - protein, 130 aa, Pisum sativum
MVFAPKSELTKKSMESYLPYVILGVLYAYLLFLSWTPETVRLIFASKYLLPELSSIGKMFSSELTLASAWIHLLVVDLFAARHIFRDGMENQIETRHSVSFCLFFCPIGILTHVITKAMTKTTRTESHGL

SEQ ID NO: 50 - protein, 248 aa, Vigna radiata
MSFSSCLSHSPLTLKPIKPCGSVGMRQNFAFSFRSNWPELCNRHIVGSRRLQGNLPRVNLSGDWSFIGGSKIVMKPNATRLLHYPKRGQMQASCFIGSQLASTAFTAGTVAVLPFYTLMVLAPNSDLTKKSMESSLPYVVLGILYAYLLYLSWTPETVRLIFASKYLLPELPGIARMFSSELTLASAWIHLLVVDLFAARHVFQDGLKNQIETRHSVSFCLFFCPIGILTHIITKAITKAATKEGHGV

SEQ ID NO: 51 - protein, 247 aa, Vigna radiata
MAFSSFFFHSPTLLKIDHLGQTKRPCGKVEKGQKFPFSVRSNGAETELCNQSQLSQRSRVRDWSFMRGSRVAMKPKILRLAPSRKVPRLYASWLSGSELASTAFTLGTTAVLPFYTLMVLAPNSQLTKKSMESSVPYIGLGVLYAYLLHLSWTPETVGLIFASKYLLPELTSIGKMFSSEMTLASAWIHLLVIDLYAARHVFLDGLENQIETRHSVSLCLFFCPIGVLTHVITKATTKSSRENKSGL

SEQ ID NO: 52 - protein, 243 aa, Trigonella foenum-graecum
MSFSSCYSHSPLPFNNKDIKLCRTVGQVKLNFPFAIRSNGVELCTRRISRCRFDLSGDWSFIGGSRIVVKPKAARSVRYTKRSQIHASWFMGSQLASTVFTWGTIAVLPFYTLMVLAPKSELTKKSMESNLPYVVLGVLYAYLLCLSWTPETVRLIFASKYLLPELTSIGKMFSSELTLASAWIHLLVVDLFAARHIFRDGMENQIETRHSVSFCLFFCPVGIVTHVITKAMTIKTRKEGHGL

SEQ ID NO: 53 - protein, 234 aa, Cichorium intybus
MAFSSCLCHHQLALKINLLTSPSKPTFALKAMNTEFYGIHIGSKLGNQWSFMKGSQAIIRPNPGSFNLHQKSSKLQASWFASMHLASDAFTLGTAAVLPFYTLMVAAPKSELTKKCMRSSIPYVVLGVLYSYLLYLSWTPDTVRLMFASKYWLPELPGVAKMFSNEMTLASAWIHLLAVDLYAARQVYHDGLEKEIETRHSVSLCLLFCPIGILVHAITKALISTYRESKTEIH

SEQ ID NO: 54 - protein, 228 aa, Allium cepa
MPLLCSCDSRIYKQATPLSNQLNKWRGLSSHAQQFIPNGSKDIVQWSFKGGSKIVIQPKISKISYHKRGSDISAYWIPTSQIASNAFTMGTVAVLPFYTLMVVAPNSKLTKRTMESSIPYVVLGMLYMYLLYLSWTPETLGYIFATKYWLPELSGISKMFSNETCTSSAWIHLLTVDLFAARQVFQDGIKNKIETRHSVSLCLLCCPIGIATHAITKALKRVSDSRSH

SEQ ID NO: 55 - protein, 249 aa, Allium cepa
MSLHYSFCNTRISHQVVHSWNAPDRYAVYAFLSARNKHDEHIGRQVAHTKSRNRVKWSFRGGSELFIQPKATRTDRQKHRSALLTSCLTSSQIAAKAFTWGTIAVLPFYTLMVVAPNAKLTKRAIESNTPYIILGAIYSYLLYLSWSPSTLRTMFASKYWLPQLSGICSMFSKEMTVASAWIHLLAVDLFAARQVYCDGILNNIETRHSISLCLLFCPIGIAIHAITKALTKYFLNYNFSEEMKLGLRS

SEQ ID NO: 56 - protein, 248 aa, Hordeum vulgare
MAAPLPSPLPRARQLHHLVDSRQEMAASPTALALALSPTTRVVVRRTPAPRVAAVSPGQLRASSWGAPLPLRPELAAAPPRPGAARRRAPLLRPRAWLSTSQIASSAFTLGTVAVLPFYTLMIAAPNANITKRTVESTAPYVALGILYAYLLYLSWTPDTIRAMFASKYWLPELPGIVRMFASEMTVASAWIHLLAVDLFAARQVYHDGIKNNIETRHSVSLCLLFCPIGIAAHALTKVLAGSTGRSH

SEQ ID NO: 57 - protein, 248 aa, unidentified
MVVAGIFIFAHSMAISSCLCHPLVLPLKDKPIGTWGNVGVDQRLTSAPRSMNAETFGRQITGVGTDLQSEWSFLGGSRVIIRPQVTKFIRHQKGFHIHASWLSGPQLVSTVFTLGTAGVLPFYTLMVFAPKAELTKKSMESSIPYVVLGVLYAYLLYLSWTPDTLRLMFASKYWLPELPGIAKMFSSEITLASAWIHLLAVDLFAASHVFQDGLQNQIETRHSVSLCLLFCPIGILTHVITKALTKSS

SEQ ID NO: 58 - protein, 235 aa, Cicer arietinum
MAFSSCFCYSSLLGLKGQKISFPIKSNCDEHYLCNKLILKSKVNLIRDWSFIGGGSRRIVVKQKVMRMASYRKAGPVYASLLSGSQLASSAFTVGTTAVLPFYTLMVLAPNSELTKKSMQSNVPYAVLGILYAYLLYLSWTPETVELIFASKYLLPELNSIGKMFSSEMTLASAWIHLLVVDLFAARQVFLDGQENQIETRHSVSLCLFFCPVGILSHVITKAMTKNTKENKHDL

SEQ ID NO: 59 - protein, 241 aa, Glycine max
MSFSSCFSHSPLTFKAMKPCGSVGKGQNFAFPIRSNGAELCKGRIVRSRVNLSGDWNFMGGSRIIVKPTATRLLLHYPKRGQMKVSCFIGSQLASTAFTAGTIAVLPFYTLMVLAPKSELTKKSMESSIPYVVLSILYAYLLYLSWTPETVRLIFASKYLLPELPGIAKMFSSEMTLASAWIHLLVIDLFAARHVFQDGLKNQIETRHSVSFCLFFCPIGILTHVITKAMTKPATKEGHGL

SEQ ID NO: 60 - protein, 241 aa, Glycine max
MYFSSCFSHSPLTLKAMKPCGSVGKGKNFAFPIRSNGAELCDGHIVRSRVNLSGDWSFIGGSRIIVKPKATRLLLHYPKRGQMQASCFIGSQLASTVFTVGTIAVLPFYTLMVLAPKSELTKKSMESSIPYVVLSILYAYLLYLSWTPETVRLIFASKYLLPELAGIAKMFSSEMTLASAWIHLLVVDLFAARHIFQDGLKNQIETRHSVSFCLFFCPIGILTHVITKSMTKPARKEGHGL

SEQ ID NO: 61 - protein, 250 aa, Glycine max
MAFSSFFSHSPLALKIDRLGQTIKPCGTVEKGQKFSFPIRSNGGELELCYQSQLNQRSRVNLIRDWSFIGGSRIVVKPNFVRLVPFRKASRVYASWLSGSQLASSAFTLGTTAVLPFYTLMVLAPNSELTRKSMESSVPYVVLGILYAYLLYHSWTPETVGLIFASKYLLPELTSIGKMFSSEMTLASAWIHLLVMDLFAARHVFLDGLENQIETRHSVSLCLFFCPIGVLSHAITKEMTKSARKNKHSL

SEQ ID NO: 62 - protein, 248 aa, Phaseolus vulgaris
MSFSSCLSHSPLTLKAIKPCGSVGKGQNFGFSFRSNEAELCNSHIAGSGRLQGNLPRVNLSGDWSFIGGSKIVVKPNATGLLPYPKRGRMQASCFIGSQLASTAFTAGTVAVLPFYTLMVLAPNSVLTKKSMDSSLPYVVLGILYAYLLYLSWTPETVRLIFASKYLLPELPGIARMFSSEMTLASAWIHLLVVDLFAARHVFQDGLKNQIETRHSVSFCLFFCPIGILTHVITKAMTKPATKEGHGV

SEQ ID NO: 63 - protein, 246 aa, Vitis vinifera
MVFSSCFCQSQISFKIDRSAVAIRPQCHTRKDQRSTFALKGMSTELFGQQVARAGAMRSSEWSFMRGSRIIIRPKVARFVFYRKGSGVYASWLANPQIASSVFTLGTAAVLPFYTLMVLAPTAELTKKSMESTIPYVVLGLLYAYLLYLSWTPDTIRLMFASKYWLPELPGMAKMFSNEMTLASAWIHLLAIDLFAARQVFQDGLENKIETRHSVSLCLLFCPIGIVTHVITKALTKSAGDTKHSM

SEQ ID NO: 64 - protein, 230 aa, Oryza sativa
MAALLLLSSAARVGVAAPLALRQQRPVVLPGGQLRTGSGAGAASAWAARPLRPELAAVSRPAVPARGRAPLFRPRAWMASSQIASSAFTWGTIAVLPFYTLMVVAPNADVTKRAVDSSAPYVALGILYAYLLYLSWTPDTLRAMFASKYWLPELTGIVRMFASEMTVASAWIHLLAVDLFAARQVYHDGIKNNIETRHSVSLCLLFCPIGIATHVLTKAYVLLTNKCAFQ

SEQ ID NO: 65 - protein, 229 aa, Triticum aestivum
MAASSPSALALSTTTRVAGSSVLLAVRRTPATRVAAVPCAQLRACSWGAPLHLRPELAAAPAPCAARCRAPLLRPRAWLSTSQIASSAFTLGTVAVLPFYTLMIAAPNANITKRAVESTAPYVALGLLYAYLLYLSWTPDTIRAMFASKYWLPELPGIVRMFASEMTVASAWIHLLAVDLFAARQVYQDGIKNNIETRHSVSLCLLFCPIGIAAHALTKVLAGSTGRSH

SEQ ID NO: 66 - protein, 232 aa, Zea mays
MAPCASPSALALSASTRVSILRLPLALRQRAEARVPGAQFRPSTACSWARPLLPELAGAVPRAGARGTGRRTQPLFRPRALTTTSQIASCAFTLGTVAVLPFYTLMVVAPNADITKRTVESGAPYVALGLLYAYLLYLSWTPDTLRAMFASKYWLPELAGIVRMFASEMTVASAWIHLLAVDLFAARQVYHDGLRNNVETRHSVSLCLLFCPVGILAHVLTKVLAGAVARSH

SEQ ID NO: 67 - protein, 246 aa, Ricinus communis
MAFSSCFCPSHIHLKTGYPRRVIRPGRPVEKDGQKFFSLRSNSTELSGRQVAKLGADLLSDWSFIGGSRIAIRPKLARAIVYRKHSGVHASWLSSYQLASTAFTLGTAAVLPFYTLMVVAPKAELTRKSMESSIPYVVLGVLYAYLLYLSWTPDTVRLMFASQYWLPELPGIAKMFSSEMTLASAWIHLLAVDLFAARQVFHDGLENEIETRHSVSLCLLFCPIGIVSHVLTKALTRSAASTRRGT

SEQ ID NO: 68 - protein, 246 aa, Populus trichocarpa
MAFSSCFCYPQFSLKNDCSGLTIRSHHIVGKDRKLFSSLRSNSIELFGQRVARVGADLHRDWNFLGGSRIIVHPKLTNFLVYRKSSGVNASWLTSTQIASSVFTLGTAAVLPFYTLMVVAPKAEVTRKSMESSIPYIVLGLLYAFLLYLSWTPDTMRLMFASQYWLPELPGIAKMFSNEMTLASAWIHLLAVDLFAARQVFNDGLENEVETRHSVSLCLLFCPIGIATHCITKALTKGSGTTTHDM

SEQ ID NO: 69 - protein, 242 aa, Malus domestica
MAFCSCFCHSPFSFKVDYGNKTIRHWSNDTSAQSFTFTLRGYNTEVLGHQVVTVESHMHKDWSFVGGSTVPIRPKLERYIPRRKCSGVYMSWLASSQIASRVFTVGTTAVLPFYALMVLAPKAQLTKVFTESSIPNVLLGVLYAYLLYLSWTPETLQLIFGSKYWLPELTGIAKMFTNEITLASAWIHLLVVDLFAARQVFSDGLQNQIETRQSVSLCLFFCPIGILTHVITKALTKTGGSL